European Patent Specification EP 3 265 481 B1, published May 1, 2024. Title: IMMUNOMODULATORY FUSION PROTEINS AND USES THEREOF. Applicant: Fred Hutchinson Cancer Research Center Oda, Shannon K. Greenberg, Philip D. Application PCT. The sequence listing filed with the application follows.

SEQUENCE LISTING (178 sequences)

SEQ ID NO: 1 - DNA, 915 bp, Artificial Sequence
  huCD200Rtm-CD28 construct
atgctgtgcccttggagaaccgccaacctgggcctgctgctgatcctgaccatcttcctggtggccgccagcagcagcctgtgcatggacgagaagcagatcacccagaactacagcaaggtgctggccgaagtgaacaccagctggcccgtgaagatggccaccaacgccgtgctgtgctgccctcctatcgccctgcggaacctgatcatcatcacctgggagatcatcctgcggggccagcccagctgtaccaaggcctaccggaaagagacaaacgagacaaaagaaacaaactgcaccgacgagcggatcacatgggtgtccagacccgaccagaacagcgacctgcagatcagacccgtggccatcacccacgacggctactaccggtgcatcatggtcacccccgatggcaacttccaccggggataccatctgcaggtgctcgtgacccccgaagtgaccctgttccagaaccggaacagaaccgccgtgtgcaaggccgtggccggaaaacctgccgcccagatctcttggatccccgagggcgattgcgccaccaagcaggaatactggtccaacggcaccgtgaccgtgaagtccacctgtcactgggaggtgcacaacgtgtccaccgtgacatgccacgtgtcccacctgaccggcaacaagagcctgtacatcgagctgctgcctgtgcctggcgccaagaagtccgccaagctgtacatcccctacatcatcctgacaatcatcattctgaccatcgtgggcttcatctggctgctgcgcagcaagcggagcagaggcggccacagcgactacatgaacatgacccctagacggcctggccccaccagaaagcactaccagccctacgcccctccccgggactttgccgcctacagaagc

SEQ ID NO: 2 - DNA, 728 bp, Artificial Sequence
  huCD200R entire extracellular domain
tgctgtgcccttggagaaccgccaacctgggcctgctgctgatcctgaccatcttcctggtggccgccagcagcagcctgtgcatggacgagaagcagatcacccagaactacagcaaggtgctggccgaagtgaacaccagctggcccgtgaagatggccaccaacgccgtgctgtgctgccctcctatcgccctgcggaacctgatcatcatcacctgggagatcatcctgcggggccagcccagctgtaccaaggcctaccggaaagagacaaacgagacaaaagaaacaaactgcaccgacgagcggatcacatgggtgtccagacccgaccagaacagcgacctgcagatcagacccgtggccatcacccacgacggctactaccggtgcatcatggtcacccccgatggcaacttccaccggggataccatctgcaggtgctcgtgacccccgaagtgaccctgttccagaaccggaacagaaccgccgtgtgcaaggccgtggccggaaaacctgccgcccagatctcttggatccccgagggcgattgcgccaccaagcaggaatactggtccaacggcaccgtgaccgtgaagtccacctgtcactgggaggtgcacaacgtgtccaccgtgacatgccacgtgtcccacctgaccggcaacaagagcctgtacatcgagctgctgcctgtgcctggcgccaagaagtccgccaagctg

SEQ ID NO: 3 - DNA, 63 bp, Artificial Sequence
  huCD200R transmembrane domain
tacatcccctacatcatcctgacaatcatcattctgaccatcgtgggcttcatctggctgctg

SEQ ID NO: 4 - DNA, 81 bp, Artificial Sequence
  CD28 transmembrane domain
ttctgggtgctggtggtggtcggaggcgtgctggcctgctacagcctgctggtcaccgtggccttcatcatcttttgggtc

SEQ ID NO: 5 - DNA, 123 bp, Artificial Sequence
  CD28 intracellular domain
cgcagcaagcggagcagaggcggccacagcgactacatgaacatgacccctagacggcctggccccaccagaaagcactaccagccctacgcccctccccgggactttgccgcctacagaagc

SEQ ID NO: 6 - DNA, 933 bp, Artificial Sequence
  huCD200R-CD28tm construct
atgctgtgcccttggagaaccgccaacctgggcctgctgctgatcctgaccatcttcctggtggccgccagcagcagcctgtgcatggacgagaagcagatcacccagaactacagcaaggtgctggccgaagtgaacaccagctggcccgtgaagatggccaccaacgccgtgctgtgctgccctcctatcgccctgcggaacctgatcatcatcacctgggagatcatcctgcggggccagcccagctgtaccaaggcctaccggaaagagacaaacgagacaaaagaaacaaactgcaccgacgagcggatcacatgggtgtccagacccgaccagaacagcgacctgcagatcagacccgtggccatcacccacgacggctactaccggtgcatcatggtcacccccgatggcaacttccaccggggataccatctgcaggtgctcgtgacccccgaagtgaccctgttccagaaccggaacagaaccgccgtgtgcaaggccgtggccggaaaacctgccgcccagatctcttggatccccgagggcgattgcgccaccaagcaggaatactggtccaacggcaccgtgaccgtgaagtccacctgtcactgggaggtgcacaacgtgtccaccgtgacatgccacgtgtcccacctgaccggcaacaagagcctgtacatcgagctgctgcctgtgcctggcgccaagaagtccgccaagctgttctgggtgctggtggtggtcggaggcgtgctggcctgctacagcctgctggtcaccgtggccttcatcatcttttgggtccgcagcaagcggagcagaggcggccacagcgactacatgaacatgacccctagacggcctggccccaccagaaagcactaccagccctacgcccctccccgggactttgccgcctacagaagc

SEQ ID NO: 7 - DNA, 942 bp, Artificial Sequence
  huCD200R-9aas-CD28Cys construct
atgctgtgcccttggagaaccgccaacctgggcctgctgctgatcctgaccatcttcctggtggccgccagcagcagcctgtgcatggacgagaagcagatcacccagaactacagcaaggtgctggccgaagtgaacaccagctggcccgtgaagatggccaccaacgccgtgctgtgctgccctcctatcgccctgcggaacctgatcatcatcacctgggagatcatcctgcggggccagcccagctgtaccaaggcctaccggaaagagacaaacgagacaaaagaaacaaactgcaccgacgagcggatcacatgggtgtccagacccgaccagaacagcgacctgcagatcagacccgtggccatcacccacgacggctactaccggtgcatcatggtcacccccgatggcaacttccaccggggataccatctgcaggtgctcgtgacccccgaagtgaccctgttccagaaccggaacagaaccgccgtgtgcaaggccgtggccggaaaacctgccgcccagatctcttggatccccgagggcgattgcgccaccaagcaggaatactggtccaacggcaccgtgaccgtgaagtccacctgtcactgggaggtgcacaacgtgtccaccgtgacatgccacgtgtcccacctgaccggcaacaagagcctgtacatcgagctgctgcctgtgtgtcccagccctctgtttcccggccctagcaagcctttctgggtgctggtggtggtcggaggcgtgctggcctgctacagcctgctggtcaccgtggccttcatcatcttttgggtccgcagcaagcggagcagaggcggccacagcgactacatgaacatgacccctagacggcctggccccaccagaaagcactaccagccctacgcccctccccgggactttgccgcctacagaagc

SEQ ID NO: 8 - DNA, 702 bp, Artificial Sequence
  huCD200R-9aas portion of extracellular domain
atgctgtgcccttggagaaccgccaacctgggcctgctgctgatcctgaccatcttcctggtggccgccagcagcagcctgtgcatggacgagaagcagatcacccagaactacagcaaggtgctggccgaagtgaacaccagctggcccgtgaagatggccaccaacgccgtgctgtgctgccctcctatcgccctgcggaacctgatcatcatcacctgggagatcatcctgcggggccagcccagctgtaccaaggcctaccggaaagagacaaacgagacaaaagaaacaaactgcaccgacgagcggatcacatgggtgtccagacccgaccagaacagcgacctgcagatcagacccgtggccatcacccacgacggctactaccggtgcatcatggtcacccccgatggcaacttccaccggggataccatctgcaggtgctcgtgacccccgaagtgaccctgttccagaaccggaacagaaccgccgtgtgcaaggccgtggccggaaaacctgccgcccagatctcttggatccccgagggcgattgcgccaccaagcaggaatactggtccaacggcaccgtgaccgtgaagtccacctgtcactgggaggtgcacaacgtgtccaccgtgacatgccacgtgtcccacctgaccggcaacaagagcctgtacatcgagctgctgcctgtg

SEQ ID NO: 9 - DNA, 36 bp, Artificial Sequence
  CD28Cys multimerization domain
tgtcccagccctctgtttcccggccctagcaagcct

SEQ ID NO: 10 - DNA, 933 bp, Artificial Sequence
  huCD200R-12aas-CD28Cys construct
atgctgtgcccttggagaaccgccaacctgggcctgctgctgatcctgaccatcttcctggtggccgccagcagcagcctgtgcatggacgagaagcagatcacccagaactacagcaaggtgctggccgaagtgaacaccagctggcccgtgaagatggccaccaacgccgtgctgtgctgccctcctatcgccctgcggaacctgatcatcatcacctgggagatcatcctgcggggccagcccagctgtaccaaggcctaccggaaagagacaaacgagacaaaagaaacaaactgcaccgacgagcggatcacatgggtgtccagacccgaccagaacagcgacctgcagatcagacccgtggccatcacccacgacggctactaccggtgcatcatggtcacccccgatggcaacttccaccggggataccatctgcaggtgctcgtgacccccgaagtgaccctgttccagaaccggaacagaaccgccgtgtgcaaggccgtggccggaaaacctgccgcccagatctcttggatccccgagggcgattgcgccaccaagcaggaatactggtccaacggcaccgtgaccgtgaagtccacctgtcactgggaggtgcacaacgtgtccaccgtgacatgccacgtgtcccacctgaccggcaacaagagcctgtacatcgagctgtgtcccagccctctgtttcccggccctagcaagcctttctgggtgctggtggtggtcggaggcgtgctggcctgctacagcctgctggtcaccgtggccttcatcatcttttgggtccgcagcaagcggagcagaggcggccacagcgactacatgaacatgacccctagacggcctggccccaccagaaagcactaccagccctacgcccctccccgggactttgccgcctacagaagc

SEQ ID NO: 11 - DNA, 693 bp, Artificial Sequence
  huCD200R-12aas portion of extracellular domain
atgctgtgcccttggagaaccgccaacctgggcctgctgctgatcctgaccatcttcctggtggccgccagcagcagcctgtgcatggacgagaagcagatcacccagaactacagcaaggtgctggccgaagtgaacaccagctggcccgtgaagatggccaccaacgccgtgctgtgctgccctcctatcgccctgcggaacctgatcatcatcacctgggagatcatcctgcggggccagcccagctgtaccaaggcctaccggaaagagacaaacgagacaaaagaaacaaactgcaccgacgagcggatcacatgggtgtccagacccgaccagaacagcgacctgcagatcagacccgtggccatcacccacgacggctactaccggtgcatcatggtcacccccgatggcaacttccaccggggataccatctgcaggtgctcgtgacccccgaagtgaccctgttccagaaccggaacagaaccgccgtgtgcaaggccgtggccggaaaacctgccgcccagatctcttggatccccgagggcgattgcgccaccaagcaggaatactggtccaacggcaccgtgaccgtgaagtccacctgtcactgggaggtgcacaacgtgtccaccgtgacatgccacgtgtcccacctgaccggcaacaagagcctgtacatcgagctg

SEQ ID NO: 12 - DNA, 945 bp, Artificial Sequence
  huCD200R-9aas-CD28Cys tm-41BBic construct
atgctgtgcccttggagaaccgccaacctgggcctgctgctgatcctgaccatcttcctggtggccgccagcagcagcctgtgcatggacgagaagcagatcacccagaactacagcaaggtgctggccgaagtgaacaccagctggcccgtgaagatggccaccaacgccgtgctgtgctgccctcctatcgccctgcggaacctgatcatcatcacctgggagatcatcctgcggggccagcccagctgtaccaaggcctaccggaaagagacaaacgagacaaaagaaacaaactgcaccgacgagcggatcacatgggtgtccagacccgaccagaacagcgacctgcagatcagacccgtggccatcacccacgacggctactaccggtgcatcatggtcacccccgatggcaacttccaccggggataccatctgcaggtgctcgtgacccccgaagtgaccctgttccagaaccggaacagaaccgccgtgtgcaaggccgtggccggaaaacctgccgcccagatctcttggatccccgagggcgattgcgccaccaagcaggaatactggtccaacggcaccgtgaccgtgaagtccacctgtcactgggaggtgcacaacgtgtccaccgtgacatgccacgtgtcccacctgaccggcaacaagagcctgtacatcgagctgctgcctgtgtgtcccagccctctgtttcccggccctagcaagcctttctgggtgctggtggtggtcggaggcgtgctggcctgctacagcctgctggtcaccgtggccttcatcatcttttgggtcaagcggggcagaaagaagctgctgtacatcttcaagcagcctttcatgcggcccgtgcagaccacccaggaagaggacggctgctcctgcagattccccgaggaagaagaaggcggctgcgagctg

SEQ ID NO: 13 - DNA, 126 bp, Artificial Sequence
  4-1BB intracellular component
aagcggggcagaaagaagctgctgtacatcttcaagcagcctttcatgcggcccgtgcagaccacccaggaagaggacggctgctcctgcagattccccgaggaagaagaaggcggctgcgagctg

SEQ ID NO: 14 - DNA, 936 bp, Artificial Sequence
  huCD200R-12aas-CD28Cys tm-41BBic construct
atgctgtgcccttggagaaccgccaacctgggcctgctgctgatcctgaccatcttcctggtggccgccagcagcagcctgtgcatggacgagaagcagatcacccagaactacagcaaggtgctggccgaagtgaacaccagctggcccgtgaagatggccaccaacgccgtgctgtgctgccctcctatcgccctgcggaacctgatcatcatcacctgggagatcatcctgcggggccagcccagctgtaccaaggcctaccggaaagagacaaacgagacaaaagaaacaaactgcaccgacgagcggatcacatgggtgtccagacccgaccagaacagcgacctgcagatcagacccgtggccatcacccacgacggctactaccggtgcatcatggtcacccccgatggcaacttccaccggggataccatctgcaggtgctcgtgacccccgaagtgaccctgttccagaaccggaacagaaccgccgtgtgcaaggccgtggccggaaaacctgccgcccagatctcttggatccccgagggcgattgcgccaccaagcaggaatactggtccaacggcaccgtgaccgtgaagtccacctgtcactgggaggtgcacaacgtgtccaccgtgacatgccacgtgtcccacctgaccggcaacaagagcctgtacatcgagctgtgtcccagccctctgtttcccggccctagcaagcctttctgggtgctggtggtggtcggaggcgtgctggcctgctacagcctgctggtcaccgtggccttcatcatcttttgggtcaagcggggcagaaagaagctgctgtacatcttcaagcagcctttcatgcggcccgtgcagaccacccaggaagaggacggctgctcctgcagattccccgaggaagaagaaggcggctgcgagctg

SEQ ID NO: 15 - DNA, 1059 bp, Artificial Sequence
  huCD200R-12aas-CD28Cys tm ic-41BBic construct
atgctgtgcccttggagaaccgccaacctgggcctgctgctgatcctgaccatcttcctggtggccgccagcagcagcctgtgcatggacgagaagcagatcacccagaactacagcaaggtgctggccgaagtgaacaccagctggcccgtgaagatggccaccaacgccgtgctgtgctgccctcctatcgccctgcggaacctgatcatcatcacctgggagatcatcctgcggggccagcccagctgtaccaaggcctaccggaaagagacaaacgagacaaaagaaacaaactgcaccgacgagcggatcacatgggtgtccagacccgaccagaacagcgacctgcagatcagacccgtggccatcacccacgacggctactaccggtgcatcatggtcacccccgatggcaacttccaccggggataccatctgcaggtgctcgtgacccccgaagtgaccctgttccagaaccggaacagaaccgccgtgtgcaaggccgtggccggaaaacctgccgcccagatctcttggatccccgagggcgattgcgccaccaagcaggaatactggtccaacggcaccgtgaccgtgaagtccacctgtcactgggaggtgcacaacgtgtccaccgtgacatgccacgtgtcccacctgaccggcaacaagagcctgtacatcgagctgtgtcccagccctctgtttcccggccctagcaagcctttctgggtgctggtggtggtcggaggcgtgctggcctgctacagcctgctggtcaccgtggccttcatcatcttttgggtccgcagcaagcggagcagaggcggccacagcgactacatgaacatgacccctagacggcctggccccaccagaaagcactaccagccctacgcccctccccgggactttgccgcctacagaagcaagcggggcagaaagaagctgctgtacatcttcaagcagcctttcatgcggcccgtgcagaccacccaggaagaggacggctgctcctgcagattccccgaggaagaagaaggcggctgcgagctg

SEQ ID NO: 16 - DNA, 1305 bp, Artificial Sequence
  huSIRPalphatm-CD28 construct
atggaacctgccggacctgctcctggcagactgggacctctgctgtgtctgctgctggccgcctcttgtgcttggagcggagtggctggcgaagaggaactgcaagtgatccagcccgacaagagcgtgctggtggccgctggcgaaaccgccaccctgagatgtacagccaccagcctgatccccgtgggccccatccagtggtttagaggcgctggccctggcagagagctgatctacaaccagaaagagggccacttccccagagtgaccaccgtgtccgacctgaccaagcggaacaacatggacttcagcatccggatcggcaacatcacccctgccgatgccggcacctactactgcgtgaagttccggaagggcagccccgacgacgtggaattcaaaagcggagccggcaccgagctgagcgtgcgggctaaaccttctgcccctgtggtgtctggacctgccgccagagctacacctcagcacaccgtgtcttttacctgcgagagccacggcttcagccccagagacatcaccctgaagtggttcaagaacggcaacgagctgtccgacttccagaccaacgtggaccctgtgggcgagagcgtgtcctacagcatccacagcaccgccaaggtggtgctgacccgcgaagatgtgcacagccaagtgatctgcgaggtggcccacgtgacactgcagggcgatcctctgagaggaaccgccaacctgtccgagacaatcagagtgccccccaccctggaagtgacccagcagcctgtgcgggccgagaaccaagtgaacgtgacctgccaagtgcggaagttctacccccagcggctgcagctgacctggctggaaaacggcaatgtgtcccggaccgagacagccagcaccgtgaccgagaacaaggatggcacctacaattggatgagctggctgctcgtgaacgtgtccgcccaccgggacgatgtgaagctgacatgccaggtggaacacgacggccagcctgccgtgtccaagagccacgatctgaaggtgtcagcccatcccaaagagcagggctccaacacagccgccgagaacaccggcagcaacgagcggaacatctacatcgtcgtgggcgtcgtgtgcaccctgctggtggcactgctgatggccgctctgtacctcgtgcgcagcaagcggagcagaggcggccacagcgactacatgaacatgacccctagacggcctggccccaccagaaagcactaccagccctacgcccctccccgggactttgccgcctacagaagc

SEQ ID NO: 17 - DNA, 1119 bp, Artificial Sequence
  huSIRP alpha entire extracellular domain
atggaacctgccggacctgctcctggcagactgggacctctgctgtgtctgctgctggccgcctcttgtgcttggagcggagtggctggcgaagaggaactgcaagtgatccagcccgacaagagcgtgctggtggccgctggcgaaaccgccaccctgagatgtacagccaccagcctgatccccgtgggccccatccagtggtttagaggcgctggccctggcagagagctgatctacaaccagaaagagggccacttccccagagtgaccaccgtgtccgacctgaccaagcggaacaacatggacttcagcatccggatcggcaacatcacccctgccgatgccggcacctactactgcgtgaagttccggaagggcagccccgacgacgtggaattcaaaagcggagccggcaccgagctgagcgtgcgggctaaaccttctgcccctgtggtgtctggacctgccgccagagctacacctcagcacaccgtgtcttttacctgcgagagccacggcttcagccccagagacatcaccctgaagtggttcaagaacggcaacgagctgtccgacttccagaccaacgtggaccctgtgggcgagagcgtgtcctacagcatccacagcaccgccaaggtggtgctgacccgcgaagatgtgcacagccaagtgatctgcgaggtggcccacgtgacactgcagggcgatcctctgagaggaaccgccaacctgtccgagacaatcagagtgccccccaccctggaagtgacccagcagcctgtgcgggccgagaaccaagtgaacgtgacctgccaagtgcggaagttctacccccagcggctgcagctgacctggctggaaaacggcaatgtgtcccggaccgagacagccagcaccgtgaccgagaacaaggatggcacctacaattggatgagctggctgctcgtgaacgtgtccgcccaccgggacgatgtgaagctgacatgccaggtggaacacgacggccagcctgccgtgtccaagagccacgatctgaaggtgtcagcccatcccaaagagcagggctccaacacagccgccgagaacaccggcagcaacgagcggaacatctac

SEQ ID NO: 18 - DNA, 63 bp, Artificial Sequence
  huSIRP alpha  transmembrane domain
atcgtcgtgggcgtcgtgtgcaccctgctggtggcactgctgatggccgctctgtacctcgtg

SEQ ID NO: 19 - DNA, 1323 bp, Artificial Sequence
  huSIRP alpha-CD28tm construct
atggaacctgccggacctgctcctggcagactgggacctctgctgtgtctgctgctggccgcctcttgtgcttggagcggagtggctggcgaagaggaactgcaagtgatccagcccgacaagagcgtgctggtggccgctggcgaaaccgccaccctgagatgtacagccaccagcctgatccccgtgggccccatccagtggtttagaggcgctggccctggcagagagctgatctacaaccagaaagagggccacttccccagagtgaccaccgtgtccgacctgaccaagcggaacaacatggacttcagcatccggatcggcaacatcacccctgccgatgccggcacctactactgcgtgaagttccggaagggcagccccgacgacgtggaattcaaaagcggagccggcaccgagctgagcgtgcgggctaaaccttctgcccctgtggtgtctggacctgccgccagagctacacctcagcacaccgtgtcttttacctgcgagagccacggcttcagccccagagacatcaccctgaagtggttcaagaacggcaacgagctgtccgacttccagaccaacgtggaccctgtgggcgagagcgtgtcctacagcatccacagcaccgccaaggtggtgctgacccgcgaagatgtgcacagccaagtgatctgcgaggtggcccacgtgacactgcagggcgatcctctgagaggaaccgccaacctgtccgagacaatcagagtgccccccaccctggaagtgacccagcagcctgtgcgggccgagaaccaagtgaacgtgacctgccaagtgcggaagttctacccccagcggctgcagctgacctggctggaaaacggcaatgtgtcccggaccgagacagccagcaccgtgaccgagaacaaggatggcacctacaattggatgagctggctgctcgtgaacgtgtccgcccaccgggacgatgtgaagctgacatgccaggtggaacacgacggccagcctgccgtgtccaagagccacgatctgaaggtgtcagcccatcccaaagagcagggctccaacacagccgccgagaacaccggcagcaacgagcggaacatctacttctgggtgctggtggtggtcggaggcgtgctggcctgctacagcctgctggtcaccgtggccttcatcatcttttgggtccgcagcaagcggagcagaggcggccacagcgactacatgaacatgacccctagacggcctggccccaccagaaagcactaccagccctacgcccctccccgggactttgccgcctacagaagc

SEQ ID NO: 20 - DNA, 1323 bp, Artificial Sequence
  huSIRP alpha 12aas-CD28Cys construct
atggaacctgccggacctgctcctggcagactgggacctctgctgtgtctgctgctggccgcctcttgtgcttggagcggagtggctggcgaagaggaactgcaagtgatccagcccgacaagagcgtgctggtggccgctggcgaaaccgccaccctgagatgtacagccaccagcctgatccccgtgggccccatccagtggtttagaggcgctggccctggcagagagctgatctacaaccagaaagagggccacttccccagagtgaccaccgtgtccgacctgaccaagcggaacaacatggacttcagcatccggatcggcaacatcacccctgccgatgccggcacctactactgcgtgaagttccggaagggcagccccgacgacgtggaattcaaaagcggagccggcaccgagctgagcgtgcgggctaaaccttctgcccctgtggtgtctggacctgccgccagagctacacctcagcacaccgtgtcttttacctgcgagagccacggcttcagccccagagacatcaccctgaagtggttcaagaacggcaacgagctgtccgacttccagaccaacgtggaccctgtgggcgagagcgtgtcctacagcatccacagcaccgccaaggtggtgctgacccgcgaagatgtgcacagccaagtgatctgcgaggtggcccacgtgacactgcagggcgatcctctgagaggaaccgccaacctgtccgagacaatcagagtgccccccaccctggaagtgacccagcagcctgtgcgggccgagaaccaagtgaacgtgacctgccaagtgcggaagttctacccccagcggctgcagctgacctggctggaaaacggcaatgtgtcccggaccgagacagccagcaccgtgaccgagaacaaggatggcacctacaattggatgagctggctgctcgtgaacgtgtccgcccaccgggacgatgtgaagctgacatgccaggtggaacacgacggccagcctgccgtgtccaagagccacgatctgaaggtgtcagcccatcccaaagagcagggctccaacacagcctgtcccagccctctgtttcccggccctagcaagcctttctgggtgctggtggtggtcggaggcgtgctggcctgctacagcctgctggtcaccgtggccttcatcatcttttgggtccgcagcaagcggagcagaggcggccacagcgactacatgaacatgacccctagacggcctggccccaccagaaagcactaccagccctacgcccctccccgggactttgccgcctacagaagc

SEQ ID NO: 21 - DNA, 1083 bp, Artificial Sequence
  huSIRP alpha 12aas portion of extracellular domain
atggaacctgccggacctgctcctggcagactgggacctctgctgtgtctgctgctggccgcctcttgtgcttggagcggagtggctggcgaagaggaactgcaagtgatccagcccgacaagagcgtgctggtggccgctggcgaaaccgccaccctgagatgtacagccaccagcctgatccccgtgggccccatccagtggtttagaggcgctggccctggcagagagctgatctacaaccagaaagagggccacttccccagagtgaccaccgtgtccgacctgaccaagcggaacaacatggacttcagcatccggatcggcaacatcacccctgccgatgccggcacctactactgcgtgaagttccggaagggcagccccgacgacgtggaattcaaaagcggagccggcaccgagctgagcgtgcgggctaaaccttctgcccctgtggtgtctggacctgccgccagagctacacctcagcacaccgtgtcttttacctgcgagagccacggcttcagccccagagacatcaccctgaagtggttcaagaacggcaacgagctgtccgacttccagaccaacgtggaccctgtgggcgagagcgtgtcctacagcatccacagcaccgccaaggtggtgctgacccgcgaagatgtgcacagccaagtgatctgcgaggtggcccacgtgacactgcagggcgatcctctgagaggaaccgccaacctgtccgagacaatcagagtgccccccaccctggaagtgacccagcagcctgtgcgggccgagaaccaagtgaacgtgacctgccaagtgcggaagttctacccccagcggctgcagctgacctggctggaaaacggcaatgtgtcccggaccgagacagccagcaccgtgaccgagaacaaggatggcacctacaattggatgagctggctgctcgtgaacgtgtccgcccaccgggacgatgtgaagctgacatgccaggtggaacacgacggccagcctgccgtgtccaagagccacgatctgaaggtgtcagcccatcccaaagagcagggctccaacacagcc

SEQ ID NO: 22 - DNA, 1326 bp, Artificial Sequence
  huSIRP alpha-12aas-CD28Cys tm-41BBic construct
atggaacctgccggacctgctcctggcagactgggacctctgctgtgtctgctgctggccgcctcttgtgcttggagcggagtggctggcgaagaggaactgcaagtgatccagcccgacaagagcgtgctggtggccgctggcgaaaccgccaccctgagatgtacagccaccagcctgatccccgtgggccccatccagtggtttagaggcgctggccctggcagagagctgatctacaaccagaaagagggccacttccccagagtgaccaccgtgtccgacctgaccaagcggaacaacatggacttcagcatccggatcggcaacatcacccctgccgatgccggcacctactactgcgtgaagttccggaagggcagccccgacgacgtggaattcaaaagcggagccggcaccgagctgagcgtgcgggctaaaccttctgcccctgtggtgtctggacctgccgccagagctacacctcagcacaccgtgtcttttacctgcgagagccacggcttcagccccagagacatcaccctgaagtggttcaagaacggcaacgagctgtccgacttccagaccaacgtggaccctgtgggcgagagcgtgtcctacagcatccacagcaccgccaaggtggtgctgacccgcgaagatgtgcacagccaagtgatctgcgaggtggcccacgtgacactgcagggcgatcctctgagaggaaccgccaacctgtccgagacaatcagagtgccccccaccctggaagtgacccagcagcctgtgcgggccgagaaccaagtgaacgtgacctgccaagtgcggaagttctacccccagcggctgcagctgacctggctggaaaacggcaatgtgtcccggaccgagacagccagcaccgtgaccgagaacaaggatggcacctacaattggatgagctggctgctcgtgaacgtgtccgcccaccgggacgatgtgaagctgacatgccaggtggaacacgacggccagcctgccgtgtccaagagccacgatctgaaggtgtcagcccatcccaaagagcagggctccaacacagcctgtcccagccctctgtttcccggccctagcaagcctttctgggtgctggtggtggtcggaggcgtgctggcctgctacagcctgctggtcaccgtggccttcatcatcttttgggtcaagcggggcagaaagaagctgctgtacatcttcaagcagcctttcatgcggcccgtgcagaccacccaggaagaggacggctgctcctgcagattccccgaggaagaagaaggcggctgcgagctg

SEQ ID NO: 23 - DNA, 1449 bp, Artificial Sequence
  huSIRP alpha-12aas-CD28Cys tm ic-41BBic construct
atggaacctgccggacctgctcctggcagactgggacctctgctgtgtctgctgctggccgcctcttgtgcttggagcggagtggctggcgaagaggaactgcaagtgatccagcccgacaagagcgtgctggtggccgctggcgaaaccgccaccctgagatgtacagccaccagcctgatccccgtgggccccatccagtggtttagaggcgctggccctggcagagagctgatctacaaccagaaagagggccacttccccagagtgaccaccgtgtccgacctgaccaagcggaacaacatggacttcagcatccggatcggcaacatcacccctgccgatgccggcacctactactgcgtgaagttccggaagggcagccccgacgacgtggaattcaaaagcggagccggcaccgagctgagcgtgcgggctaaaccttctgcccctgtggtgtctggacctgccgccagagctacacctcagcacaccgtgtcttttacctgcgagagccacggcttcagccccagagacatcaccctgaagtggttcaagaacggcaacgagctgtccgacttccagaccaacgtggaccctgtgggcgagagcgtgtcctacagcatccacagcaccgccaaggtggtgctgacccgcgaagatgtgcacagccaagtgatctgcgaggtggcccacgtgacactgcagggcgatcctctgagaggaaccgccaacctgtccgagacaatcagagtgccccccaccctggaagtgacccagcagcctgtgcgggccgagaaccaagtgaacgtgacctgccaagtgcggaagttctacccccagcggctgcagctgacctggctggaaaacggcaatgtgtcccggaccgagacagccagcaccgtgaccgagaacaaggatggcacctacaattggatgagctggctgctcgtgaacgtgtccgcccaccgggacgatgtgaagctgacatgccaggtggaacacgacggccagcctgccgtgtccaagagccacgatctgaaggtgtcagcccatcccaaagagcagggctccaacacagcctgtcccagccctctgtttcccggccctagcaagcctttctgggtgctggtggtggtcggaggcgtgctggcctgctacagcctgctggtcaccgtggccttcatcatcttttgggtccgcagcaagcggagcagaggcggccacagcgactacatgaacatgacccctagacggcctggccccaccagaaagcactaccagccctacgcccctccccgggactttgccgcctacagaagcaagcggggcagaaagaagctgctgtacatcttcaagcagcctttcatgcggcccgtgcagaccacccaggaagaggacggctgctcctgcagattccccgaggaagaagaaggcggctgcgagctg

SEQ ID NO: 24 - protein, 305 aa, Artificial Sequence
  huCD200Rtm-CD28 protein
MLCPWRTANLGLLLILTIFLVAASSSLCMDEKQITQNYSKVLAEVNTSWPVKMATNAVLCCPPIALRNLIIITWEIILRGQPSCTKAYRKETNETKETNCTDERITWVSRPDQNSDLQIRPVAITHDGYYRCIMVTPDGNFHRGYHLQVLVTPEVTLFQNRNRTAVCKAVAGKPAAQISWIPEGDCATKQEYWSNGTVTVKSTCHWEVHNVSTVTCHVSHLTGNKSLYIELLPVPGAKKSAKLYIPYIILTIIILTIVGFIWLLRSKRSRGGHSDYMNMTPRRPGPTRKHYQPYAPPRDFAAYRS

SEQ ID NO: 25 - protein, 243 aa, Artificial Sequence
  huCD200R entire extracellular domain
MLCPWRTANLGLLLILTIFLVAASSSLCMDEKQITQNYSKVLAEVNTSWPVKMATNAVLCCPPIALRNLIIITWEIILRGQPSCTKAYRKETNETKETNCTDERITWVSRPDQNSDLQIRPVAITHDGYYRCIMVTPDGNFHRGYHLQVLVTPEVTLFQNRNRTAVCKAVAGKPAAQISWIPEGDCATKQEYWSNGTVTVKSTCHWEVHNVSTVTCHVSHLTGNKSLYIELLPVPGAKKSAKL

SEQ ID NO: 26 - protein, 21 aa, Artificial Sequence
  huCD200R transmembrane domain
YIPYIILTIIILTIVGFIWLL

SEQ ID NO: 27 - protein, 27 aa, Artificial Sequence
  CD28 transmembrane domain protein
FWVLVVVGGVLACYSLLVTVAFIIFWV

SEQ ID NO: 28 - protein, 41 aa, Artificial Sequence
  CD28 intracellular domain protein
RSKRSRGGHSDYMNMTPRRPGPTRKHYQPYAPPRDFAAYRS

SEQ ID NO: 29 - protein, 311 aa, Artificial Sequence
  huCD200R-CD28tm protein
MLCPWRTANLGLLLILTIFLVAASSSLCMDEKQITQNYSKVLAEVNTSWPVKMATNAVLCCPPIALRNLIIITWEIILRGQPSCTKAYRKETNETKETNCTDERITWVSRPDQNSDLQIRPVAITHDGYYRCIMVTPDGNFHRGYHLQVLVTPEVTLFQNRNRTAVCKAVAGKPAAQISWIPEGDCATKQEYWSNGTVTVKSTCHWEVHNVSTVTCHVSHLTGNKSLYIELLPVPGAKKSAKLFWVLVVVGGVLACYSLLVTVAFIIFWVRSKRSRGGHSDYMNMTPRRPGPTRKHYQPYAPPRDFAAYRS

SEQ ID NO: 30 - protein, 314 aa, Artificial Sequence
  huCD200R-9aas-CD28Cys protein
MLCPWRTANLGLLLILTIFLVAASSSLCMDEKQITQNYSKVLAEVNTSWPVKMATNAVLCCPPIALRNLIIITWEIILRGQPSCTKAYRKETNETKETNCTDERITWVSRPDQNSDLQIRPVAITHDGYYRCIMVTPDGNFHRGYHLQVLVTPEVTLFQNRNRTAVCKAVAGKPAAQISWIPEGDCATKQEYWSNGTVTVKSTCHWEVHNVSTVTCHVSHLTGNKSLYIELLPVCPSPLFPGPSKPFWVLVVVGGVLACYSLLVTVAFIIFWVRSKRSRGGHSDYMNMTPRRPGPTRKHYQPYAPPRDFAAYRS

SEQ ID NO: 31 - protein, 234 aa, Artificial Sequence
  huCD200R-9aas protein
MLCPWRTANLGLLLILTIFLVAASSSLCMDEKQITQNYSKVLAEVNTSWPVKMATNAVLCCPPIALRNLIIITWEIILRGQPSCTKAYRKETNETKETNCTDERITWVSRPDQNSDLQIRPVAITHDGYYRCIMVTPDGNFHRGYHLQVLVTPEVTLFQNRNRTAVCKAVAGKPAAQISWIPEGDCATKQEYWSNGTVTVKSTCHWEVHNVSTVTCHVSHLTGNKSLYIELLPV

SEQ ID NO: 32 - protein, 12 aa, Artificial Sequence
  CD28Cys (extracellular portion) protein
CPSPLFPGPSKP

SEQ ID NO: 33 - protein, 311 aa, Artificial Sequence
  huCD200R-12aas-CD28Cys protein
MLCPWRTANLGLLLILTIFLVAASSSLCMDEKQITQNYSKVLAEVNTSWPVKMATNAVLCCPPIALRNLIIITWEIILRGQPSCTKAYRKETNETKETNCTDERITWVSRPDQNSDLQIRPVAITHDGYYRCIMVTPDGNFHRGYHLQVLVTPEVTLFQNRNRTAVCKAVAGKPAAQISWIPEGDCATKQEYWSNGTVTVKSTCHWEVHNVSTVTCHVSHLTGNKSLYIELCPSPLFPGPSKPFWVLVVVGGVLACYSLLVTVAFIIFWVRSKRSRGGHSDYMNMTPRRPGPTRKHYQPYAPPRDFAAYRS

SEQ ID NO: 34 - protein, 231 aa, Artificial Sequence
  huCD200R-12aas protein
MLCPWRTANLGLLLILTIFLVAASSSLCMDEKQITQNYSKVLAEVNTSWPVKMATNAVLCCPPIALRNLIIITWEIILRGQPSCTKAYRKETNETKETNCTDERITWVSRPDQNSDLQIRPVAITHDGYYRCIMVTPDGNFHRGYHLQVLVTPEVTLFQNRNRTAVCKAVAGKPAAQISWIPEGDCATKQEYWSNGTVTVKSTCHWEVHNVSTVTCHVSHLTGNKSLYIEL

SEQ ID NO: 35 - protein, 315 aa, Artificial Sequence
  huCD200R-9aas-CD28Cys tm-41BBic protein
MLCPWRTANLGLLLILTIFLVAASSSLCMDEKQITQNYSKVLAEVNTSWPVKMATNAVLCCPPIALRNLIIITWEIILRGQPSCTKAYRKETNETKETNCTDERITWVSRPDQNSDLQIRPVAITHDGYYRCIMVTPDGNFHRGYHLQVLVTPEVTLFQNRNRTAVCKAVAGKPAAQISWIPEGDCATKQEYWSNGTVTVKSTCHWEVHNVSTVTCHVSHLTGNKSLYIELLPVCPSPLFPGPSKPFWVLVVVGGVLACYSLLVTVAFIIFWVKRGRKKLLYIFKQPFMRPVQTTQEEDGCSCRFPEEEEGGCEL

SEQ ID NO: 36 - protein, 42 aa, Artificial Sequence
  4-1BB intracellular component protein
KRGRKKLLYIFKQPFMRPVQTTQEEDGCSCRFPEEEEGGCEL

SEQ ID NO: 37 - protein, 312 aa, Artificial Sequence
  huCD200R-12aas-CD28Cys tm-41BBic protein
MLCPWRTANLGLLLILTIFLVAASSSLCMDEKQITQNYSKVLAEVNTSWPVKMATNAVLCCPPIALRNLIIITWEIILRGQPSCTKAYRKETNETKETNCTDERITWVSRPDQNSDLQIRPVAITHDGYYRCIMVTPDGNFHRGYHLQVLVTPEVTLFQNRNRTAVCKAVAGKPAAQISWIPEGDCATKQEYWSNGTVTVKSTCHWEVHNVSTVTCHVSHLTGNKSLYIELCPSPLFPGPSKPFWVLVVVGGVLACYSLLVTVAFIIFWVKRGRKKLLYIFKQPFMRPVQTTQEEDGCSCRFPEEEEGGCEL

SEQ ID NO: 38 - protein, 353 aa, Artificial Sequence
  huCD200R-12aas-CD28Cys tm ic-41BBic protein
MLCPWRTANLGLLLILTIFLVAASSSLCMDEKQITQNYSKVLAEVNTSWPVKMATNAVLCCPPIALRNLIIITWEIILRGQPSCTKAYRKETNETKETNCTDERITWVSRPDQNSDLQIRPVAITHDGYYRCIMVTPDGNFHRGYHLQVLVTPEVTLFQNRNRTAVCKAVAGKPAAQISWIPEGDCATKQEYWSNGTVTVKSTCHWEVHNVSTVTCHVSHLTGNKSLYIELCPSPLFPGPSKPFWVLVVVGGVLACYSLLVTVAFIIFWVRSKRSRGGHSDYMNMTPRRPGPTRKHYQPYAPPRDFAAYRSKRGRKKLLYIFKQPFMRPVQTTQEEDGCSCRFPEEEEGGCEL

SEQ ID NO: 39 - protein, 435 aa, Artificial Sequence
  huSIRP alpha tm-CD28 protein
MEPAGPAPGRLGPLLCLLLAASCAWSGVAGEEELQVIQPDKSVLVAAGETATLRCTATSLIPVGPIQWFRGAGPGRELIYNQKEGHFPRVTTVSDLTKRNNMDFSIRIGNITPADAGTYYCVKFRKGSPDDVEFKSGAGTELSVRAKPSAPVVSGPAARATPQHTVSFTCESHGFSPRDITLKWFKNGNELSDFQTNVDPVGESVSYSIHSTAKVVLTREDVHSQVICEVAHVTLQGDPLRGTANLSETIRVPPTLEVTQQPVRAENQVNVTCQVRKFYPQRLQLTWLENGNVSRTETASTVTENKDGTYNWMSWLLVNVSAHRDDVKLTCQVEHDGQPAVSKSHDLKVSAHPKEQGSNTAAENTGSNERNIYIVVGVVCTLLVALLMAALYLVRSKRSRGGHSDYMNMTPRRPGPTRKHYQPYAPPRDFAAYRS

SEQ ID NO: 40 - protein, 373 aa, Artificial Sequence
  huSIRP alpha entire extracellular domain protein
MEPAGPAPGRLGPLLCLLLAASCAWSGVAGEEELQVIQPDKSVLVAAGETATLRCTATSLIPVGPIQWFRGAGPGRELIYNQKEGHFPRVTTVSDLTKRNNMDFSIRIGNITPADAGTYYCVKFRKGSPDDVEFKSGAGTELSVRAKPSAPVVSGPAARATPQHTVSFTCESHGFSPRDITLKWFKNGNELSDFQTNVDPVGESVSYSIHSTAKVVLTREDVHSQVICEVAHVTLQGDPLRGTANLSETIRVPPTLEVTQQPVRAENQVNVTCQVRKFYPQRLQLTWLENGNVSRTETASTVTENKDGTYNWMSWLLVNVSAHRDDVKLTCQVEHDGQPAVSKSHDLKVSAHPKEQGSNTAAENTGSNERNIY

SEQ ID NO: 41 - protein, 21 aa, Artificial Sequence
  huSIRP alpha transmembrane domain protein
IVVGVVCTLLVALLMAALYLV

SEQ ID NO: 42 - protein, 441 aa, Artificial Sequence
  huSIRP alpha -CD28tm protein
MEPAGPAPGRLGPLLCLLLAASCAWSGVAGEEELQVIQPDKSVLVAAGETATLRCTATSLIPVGPIQWFRGAGPGRELIYNQKEGHFPRVTTVSDLTKRNNMDFSIRIGNITPADAGTYYCVKFRKGSPDDVEFKSGAGTELSVRAKPSAPVVSGPAARATPQHTVSFTCESHGFSPRDITLKWFKNGNELSDFQTNVDPVGESVSYSIHSTAKVVLTREDVHSQVICEVAHVTLQGDPLRGTANLSETIRVPPTLEVTQQPVRAENQVNVTCQVRKFYPQRLQLTWLENGNVSRTETASTVTENKDGTYNWMSWLLVNVSAHRDDVKLTCQVEHDGQPAVSKSHDLKVSAHPKEQGSNTAAENTGSNERNIYFWVLVVVGGVLACYSLLVTVAFIIFWVRSKRSRGGHSDYMNMTPRRPGPTRKHYQPYAPPRDFAAYRS

SEQ ID NO: 43 - protein, 441 aa, Artificial Sequence
  huSIRP alpha-12aas-CD28Cys protein
MEPAGPAPGRLGPLLCLLLAASCAWSGVAGEEELQVIQPDKSVLVAAGETATLRCTATSLIPVGPIQWFRGAGPGRELIYNQKEGHFPRVTTVSDLTKRNNMDFSIRIGNITPADAGTYYCVKFRKGSPDDVEFKSGAGTELSVRAKPSAPVVSGPAARATPQHTVSFTCESHGFSPRDITLKWFKNGNELSDFQTNVDPVGESVSYSIHSTAKVVLTREDVHSQVICEVAHVTLQGDPLRGTANLSETIRVPPTLEVTQQPVRAENQVNVTCQVRKFYPQRLQLTWLENGNVSRTETASTVTENKDGTYNWMSWLLVNVSAHRDDVKLTCQVEHDGQPAVSKSHDLKVSAHPKEQGSNTACPSPLFPGPSKPFWVLVVVGGVLACYSLLVTVAFIIFWVRSKRSRGGHSDYMNMTPRRPGPTRKHYQPYAPPRDFAAYRS

SEQ ID NO: 44 - protein, 361 aa, Artificial Sequence
  huSIRP alpha-12aas protein
MEPAGPAPGRLGPLLCLLLAASCAWSGVAGEEELQVIQPDKSVLVAAGETATLRCTATSLIPVGPIQWFRGAGPGRELIYNQKEGHFPRVTTVSDLTKRNNMDFSIRIGNITPADAGTYYCVKFRKGSPDDVEFKSGAGTELSVRAKPSAPVVSGPAARATPQHTVSFTCESHGFSPRDITLKWFKNGNELSDFQTNVDPVGESVSYSIHSTAKVVLTREDVHSQVICEVAHVTLQGDPLRGTANLSETIRVPPTLEVTQQPVRAENQVNVTCQVRKFYPQRLQLTWLENGNVSRTETASTVTENKDGTYNWMSWLLVNVSAHRDDVKLTCQVEHDGQPAVSKSHDLKVSAHPKEQGSNTA

SEQ ID NO: 45 - protein, 442 aa, Artificial Sequence
  huSIRP alpha-12aas-CD28Cys tm-41BBic protein
MEPAGPAPGRLGPLLCLLLAASCAWSGVAGEEELQVIQPDKSVLVAAGETATLRCTATSLIPVGPIQWFRGAGPGRELIYNQKEGHFPRVTTVSDLTKRNNMDFSIRIGNITPADAGTYYCVKFRKGSPDDVEFKSGAGTELSVRAKPSAPVVSGPAARATPQHTVSFTCESHGFSPRDITLKWFKNGNELSDFQTNVDPVGESVSYSIHSTAKVVLTREDVHSQVICEVAHVTLQGDPLRGTANLSETIRVPPTLEVTQQPVRAENQVNVTCQVRKFYPQRLQLTWLENGNVSRTETASTVTENKDGTYNWMSWLLVNVSAHRDDVKLTCQVEHDGQPAVSKSHDLKVSAHPKEQGSNTACPSPLFPGPSKPFWVLVVVGGVLACYSLLVTVAFIIFWVKRGRKKLLYIFKQPFMRPVQTTQEEDGCSCRFPEEEEGGCEL

SEQ ID NO: 46 - protein, 483 aa, Artificial Sequence
  huSIRP alpha-12aas-CD28Cys tm ic-41BBic protein
MEPAGPAPGRLGPLLCLLLAASCAWSGVAGEEELQVIQPDKSVLVAAGETATLRCTATSLIPVGPIQWFRGAGPGRELIYNQKEGHFPRVTTVSDLTKRNNMDFSIRIGNITPADAGTYYCVKFRKGSPDDVEFKSGAGTELSVRAKPSAPVVSGPAARATPQHTVSFTCESHGFSPRDITLKWFKNGNELSDFQTNVDPVGESVSYSIHSTAKVVLTREDVHSQVICEVAHVTLQGDPLRGTANLSETIRVPPTLEVTQQPVRAENQVNVTCQVRKFYPQRLQLTWLENGNVSRTETASTVTENKDGTYNWMSWLLVNVSAHRDDVKLTCQVEHDGQPAVSKSHDLKVSAHPKEQGSNTACPSPLFPGPSKPFWVLVVVGGVLACYSLLVTVAFIIFWVRSKRSRGGHSDYMNMTPRRPGPTRKHYQPYAPPRDFAAYRSKRGRKKLLYIFKQPFMRPVQTTQEEDGCSCRFPEEEEGGCEL

SEQ ID NO: 47 - DNA, 900 bp, Artificial Sequence
  muCD200Rtm-CD28
atgttctgcttctggcggacaagcgccctggccgtgctgctgatctggggagtgtttgtggccggcagcagctgcaccgacaagaaccagaccacccagaacaacagcagcagccccctgacccaagtgaacaccaccgtgtccgtgcagatcggcaccaaggccctgctgtgctgtttcagcatccctctgaccaaggctgtgctgatcacctggatcatcaagctgagaggcctgcccagctgcacaatcgcctacaaggtggacaccaagaccaacgagacaagctgcctgggcagaaacatcacctgggccagcaccccagaccacagccctgagctgcagatcagcgccgtgacactgcagcacgagggcacctacacatgcgagacagtgacccccgagggcaacttcgagaagaactacgatctgcaggtgctggtgccccccgaagtgacctacttccccgagaagaatagaagcgccgtgtgcgaggccatggctggcaaacctgccgcccagatctcttggagccctgacggcgactgtgtgaccaccagcgagagccacagcaacggcacagtgaccgtgcggagcacctgtcactgggagcagaacaacgtgtccgacgtgtcctgcatcgtgtcccacctgaccggcaaccagagcctgagcatcgagctgagcagaggcggaaaccagtccctgaggccctacatcccttacatcatccccagcatcatcatcctgatcatcatcggctgcatctgcctgctgaacagcagaagaaacagaggcggccagagcgactacatgaacatgacccccagaaggcctggcctgaccagaaagccctaccagccttacgcccctgccagagacttcgccgcctacagacct

SEQ ID NO: 48 - DNA, 918 bp, Artificial Sequence
  muCD200R-CD28tm
atgttctgcttctggcggacaagcgccctggccgtgctgctgatctggggagtgtttgtggccggcagcagctgcaccgacaagaaccagaccacccagaacaacagcagcagccccctgacccaagtgaacaccaccgtgtccgtgcagatcggcaccaaggccctgctgtgctgtttcagcatccctctgaccaaggctgtgctgatcacctggatcatcaagctgagaggcctgcccagctgcacaatcgcctacaaggtggacaccaagaccaacgagacaagctgcctgggcagaaacatcacctgggccagcaccccagaccacagccctgagctgcagatcagcgccgtgacactgcagcacgagggcacctacacatgcgagacagtgacccccgagggcaacttcgagaagaactacgatctgcaggtgctggtgccccccgaagtgacctacttccccgagaagaatagaagcgccgtgtgcgaggccatggctggcaaacctgccgcccagatctcttggagccctgacggcgactgtgtgaccaccagcgagagccacagcaacggcacagtgaccgtgcggagcacctgtcactgggagcagaacaacgtgtccgacgtgtcctgcatcgtgtcccacctgaccggcaaccagagcctgagcatcgagctgagcagaggcggaaaccagtccctgaggcccttctgggccctggtggtggtggccggcgtgctgttttgttacggcctgctcgtgaccgtggccctgtgcgtgatctggaccaacagcagaagaaacagaggcggccagagcgactacatgaacatgacccccagaaggcctggcctgaccagaaagccctaccagccttacgcccctgccagagacttcgccgcctacagacct

SEQ ID NO: 49 - DNA, 945 bp, Artificial Sequence
  muCD200R-CD28Cys
atgttctgcttctggcggacaagcgccctggccgtgctgctgatctggggagtgtttgtggccggcagcagctgcaccgacaagaaccagaccacccagaacaacagcagcagccccctgacccaagtgaacaccaccgtgtccgtgcagatcggcaccaaggccctgctgtgctgtttcagcatccctctgaccaaggctgtgctgatcacctggatcatcaagctgagaggcctgcccagctgcacaatcgcctacaaggtggacaccaagaccaacgagacaagctgcctgggcagaaacatcacctgggccagcaccccagaccacagccctgagctgcagatcagcgccgtgacactgcagcacgagggcacctacacatgcgagacagtgacccccgagggcaacttcgagaagaactacgatctgcaggtgctggtgccccccgaagtgacctacttccccgagaagaatagaagcgccgtgtgcgaggccatggctggcaaacctgccgcccagatctcttggagccctgacggcgactgtgtgaccaccagcgagagccacagcaacggcacagtgaccgtgcggagcacctgtcactgggagcagaacaacgtgtccgacgtgtcctgcatcgtgtcccacctgaccggcaaccagagcctgagcatcgagctgagcagaggcggaaaccagtccctgaggccctgccacacccagagcagccccaagctgttctgggccctggtggtggtggccggcgtgctgttttgttacggcctgctcgtgaccgtggccctgtgcgtgatctggaccaacagcagaagaaacagaggcggccagagcgactacatgaacatgacccccagaaggcctggcctgaccagaaagccctaccagccttacgcccctgccagagacttcgccgcctacagacct

SEQ ID NO: 50 - DNA, 936 bp, Artificial Sequence
  muCD200R-3aas-CD28Cys
atgttctgcttctggcggacaagcgccctggccgtgctgctgatctggggagtgtttgtggccggcagcagctgcaccgacaagaaccagaccacccagaacaacagcagcagccccctgacccaagtgaacaccaccgtgtccgtgcagatcggcaccaaggccctgctgtgctgtttcagcatccctctgaccaaggctgtgctgatcacctggatcatcaagctgagaggcctgcccagctgcacaatcgcctacaaggtggacaccaagaccaacgagacaagctgcctgggcagaaacatcacctgggccagcaccccagaccacagccctgagctgcagatcagcgccgtgacactgcagcacgagggcacctacacatgcgagacagtgacccccgagggcaacttcgagaagaactacgatctgcaggtgctggtgccccccgaagtgacctacttccccgagaagaatagaagcgccgtgtgcgaggccatggctggcaaacctgccgcccagatctcttggagccctgacggcgactgtgtgaccaccagcgagagccacagcaacggcacagtgaccgtgcggagcacctgtcactgggagcagaacaacgtgtccgacgtgtcctgcatcgtgtcccacctgaccggcaaccagagcctgagcatcgagctgagcagaggcggaaaccagtcctgccacacccagagcagccccaagctgttctgggccctggtggtggtggccggcgtgctgttttgttacggcctgctcgtgaccgtggccctgtgcgtgatctggaccaacagcagaagaaacagaggcggccagagcgactacatgaacatgacccccagaaggcctggcctgaccagaaagccctaccagccttacgcccctgccagagacttcgccgcctacagacct

SEQ ID NO: 51 - DNA, 918 bp, Artificial Sequence
  muCD200R-9aas-CD28Cys
atgttctgcttctggcggacaagcgccctggccgtgctgctgatctggggagtgtttgtggccggcagcagctgcaccgacaagaaccagaccacccagaacaacagcagcagccccctgacccaagtgaacaccaccgtgtccgtgcagatcggcaccaaggccctgctgtgctgtttcagcatccctctgaccaaggctgtgctgatcacctggatcatcaagctgagaggcctgcccagctgcacaatcgcctacaaggtggacaccaagaccaacgagacaagctgcctgggcagaaacatcacctgggccagcaccccagaccacagccctgagctgcagatcagcgccgtgacactgcagcacgagggcacctacacatgcgagacagtgacccccgagggcaacttcgagaagaactacgatctgcaggtgctggtgccccccgaagtgacctacttccccgagaagaatagaagcgccgtgtgcgaggccatggctggcaaacctgccgcccagatctcttggagccctgacggcgactgtgtgaccaccagcgagagccacagcaacggcacagtgaccgtgcggagcacctgtcactgggagcagaacaacgtgtccgacgtgtcctgcatcgtgtcccacctgaccggcaaccagagcctgagcatcgagctgagctgccacacccagagcagccccaagctgttctgggccctggtggtggtggccggcgtgctgttttgttacggcctgctcgtgaccgtggccctgtgcgtgatctggaccaacagcagaagaaacagaggcggccagagcgactacatgaacatgacccccagaaggcctggcctgaccagaaagccctaccagccttacgcccctgccagagacttcgccgcctacagacct

SEQ ID NO: 52 - DNA, 939 bp, Artificial Sequence
  muCD200R-9aas-CD28Cys tm-41BBic
atgttctgcttctggcggacaagcgccctggccgtgctgctgatctggggagtgtttgtggccggcagcagctgcaccgacaagaaccagaccacccagaacaacagcagcagccccctgacccaagtgaacaccaccgtgtccgtgcagatcggcaccaaggccctgctgtgctgtttcagcatccctctgaccaaggctgtgctgatcacctggatcatcaagctgagaggcctgcccagctgcacaatcgcctacaaggtggacaccaagaccaacgagacaagctgcctgggcagaaacatcacctgggccagcaccccagaccacagccctgagctgcagatcagcgccgtgacactgcagcacgagggcacctacacatgcgagacagtgacccccgagggcaacttcgagaagaactacgatctgcaggtgctggtgccccccgaagtgacctacttccccgagaagaatagaagcgccgtgtgcgaggccatggctggcaaacctgccgcccagatctcttggagccctgacggcgactgtgtgaccaccagcgagagccacagcaacggcacagtgaccgtgcggagcacctgtcactgggagcagaacaacgtgtccgacgtgtcctgcatcgtgtcccacctgaccggcaaccagagcctgagcatcgagctgagctgccacacccagagcagccccaagctgttctgggccctggtggtggtggccggcgtgctgttttgttacggcctgctcgtgaccgtggccctgtgcgtgatctggaccagcgtgctgaagtggatcagaaagaagttcccccacatcttcaagcagcccttcaagaaaaccaccggcgctgcccaggaagaggacgcctgcagctgtagatgccctcaggaagaagaaggcggcggaggcggctacgagctg

SEQ ID NO: 53 - DNA, 1062 bp, Artificial Sequence
  muCD200R-9aas-CD28Cys tm ic-41BBic
atgttctgcttctggcggacaagcgccctggccgtgctgctgatctggggagtgtttgtggccggcagcagctgcaccgacaagaaccagaccacccagaacaacagcagcagccccctgacccaagtgaacaccaccgtgtccgtgcagatcggcaccaaggccctgctgtgctgtttcagcatccctctgaccaaggctgtgctgatcacctggatcatcaagctgagaggcctgcccagctgcacaatcgcctacaaggtggacaccaagaccaacgagacaagctgcctgggcagaaacatcacctgggccagcaccccagaccacagccctgagctgcagatcagcgccgtgacactgcagcacgagggcacctacacatgcgagacagtgacccccgagggcaacttcgagaagaactacgatctgcaggtgctggtgccccccgaagtgacctacttccccgagaagaatagaagcgccgtgtgcgaggccatggctggcaaacctgccgcccagatctcttggagccctgacggcgactgtgtgaccaccagcgagagccacagcaacggcacagtgaccgtgcggagcacctgtcactgggagcagaacaacgtgtccgacgtgtcctgcatcgtgtcccacctgaccggcaaccagagcctgagcatcgagctgagctgccacacccagagcagccccaagctgttctgggccctggtggtggtggccggcgtgctgttttgttacggcctgctcgtgaccgtggccctgtgcgtgatctggaccaacagcagaagaaacagaggcggccagagcgactacatgaacatgacccccagaaggcctggcctgaccagaaagccctaccagccttacgcccctgccagagacttcgccgcctacagacctagcgtgctgaagtggatcagaaagaagttcccccacatcttcaagcagcccttcaagaaaaccaccggcgctgcccaggaagaggacgcctgcagctgtagatgccctcaggaagaagaaggcggcggaggcggctacgagctg

SEQ ID NO: 54 - DNA, 1305 bp, Artificial Sequence
  muSIRP alpha  tm-CD28
atggaacctgctggacctgcccctggcagactgggacctctgctgctgtgcctgctgctgagcgccagctgtttctgtaccggcgccaccggcaaagaactgaaagtgacccagcccgagaagtccgtgtctgtggccgctggcgacagcaccgtgctgaactgtaccctgaccagcctgctgcccgtgggccccatcagatggtatagaggcgtgggccctagcagactgctgatctacagcttcgctggcgagtacgtgcccagaatcagaaacgtgtccgacaccaccaagcggaacaacatggacttcagcatcaggatcagcaacgtgacccctgccgacgccggcatctactactgcgtgaagttccagaagggcagcagcgagcccgacaccgagattcagtctggcggcggaaccgaggtgtacgtgctggctaagcccagccctcctgaggtgtccggccctgctgatagaggcatccccgaccagaaagtgaacttcacatgcaagagccacggcttcagccccagaaacatcaccctgaagtggttcaaggacggccaggaactgcaccccctggaaaccaccgtgaaccccagcggcaagaacgtgtcctacaacatcagctccaccgtgcgggtggtgctgaacagcatggacgtgaacagcaaagtgatctgcgaggtggcccacatcacactggacagaagccccctgagaggaatcgccaacctgagcaacttcatcagagtgtccccaaccgtgaaagtgacacagcagagccccaccagcatgaaccaagtgaacctgacctgcagagccgagagattctaccccgaggacctgcagctgatctggctggaaaacggcaacgtgtccagaaacgacacccccaagaacctgacaaagaacaccgacggcacctacaactacacctccctgtttctcgtgaactcctccgcccaccgcgaggacgtggtgttcacgtgccaagtgaagcacgaccagcagcccgccatcaccagaaaccacacagtgctgggcttcgcccacagcagcgaccagggcagcatgcagaccttccccgacaacaacgccacccacaactggaacgtgttcatcggcgtgggcgtggcctgtgctctgctggtggtgctgctgatggccgccctgtataacagcagaagaaacagaggcggccagagcgactacatgaacatgacccccagaaggcctggcctgaccagaaagccctaccagccttacgcccctgccagagacttcgccgcctacagacct

SEQ ID NO: 55 - DNA, 1323 bp, Artificial Sequence
  muSIRP alpha-CD28tm
atggaacctgctggacctgcccctggcagactgggacctctgctgctgtgcctgctgctgagcgccagctgtttctgtaccggcgccaccggcaaagaactgaaagtgacccagcccgagaagtccgtgtctgtggccgctggcgacagcaccgtgctgaactgtaccctgaccagcctgctgcccgtgggccccatcagatggtatagaggcgtgggccctagcagactgctgatctacagcttcgctggcgagtacgtgcccagaatcagaaacgtgtccgacaccaccaagcggaacaacatggacttcagcatcaggatcagcaacgtgacccctgccgacgccggcatctactactgcgtgaagttccagaagggcagcagcgagcccgacaccgagattcagtctggcggcggaaccgaggtgtacgtgctggctaagcccagccctcctgaggtgtccggccctgctgatagaggcatccccgaccagaaagtgaacttcacatgcaagagccacggcttcagccccagaaacatcaccctgaagtggttcaaggacggccaggaactgcaccccctggaaaccaccgtgaaccccagcggcaagaacgtgtcctacaacatcagctccaccgtgcgggtggtgctgaacagcatggacgtgaacagcaaagtgatctgcgaggtggcccacatcacactggacagaagccccctgagaggaatcgccaacctgagcaacttcatcagagtgtccccaaccgtgaaagtgacacagcagagccccaccagcatgaaccaagtgaacctgacctgcagagccgagagattctaccccgaggacctgcagctgatctggctggaaaacggcaacgtgtccagaaacgacacccccaagaacctgacaaagaacaccgacggcacctacaactacacctccctgtttctcgtgaactcctccgcccaccgcgaggacgtggtgttcacgtgccaagtgaagcacgaccagcagcccgccatcaccagaaaccacacagtgctgggcttcgcccacagcagcgaccagggcagcatgcagaccttccccgacaacaacgccacccacaactggaacttctgggccctggtggtggtggccggcgtgctgttttgttacggcctgctcgtgaccgtggccctgtgcgtgatctggaccaacagcagaagaaacagaggcggccagagcgactacatgaacatgacccccagaaggcctggcctgaccagaaagccctaccagccttacgcccctgccagagacttcgccgcctacagacct

SEQ ID NO: 56 - DNA, 1350 bp, Artificial Sequence
  muSIRP alpha-CD28cys
atggaacctgctggacctgcccctggcagactgggacctctgctgctgtgcctgctgctgagcgccagctgtttctgtaccggcgccaccggcaaagaactgaaagtgacccagcccgagaagtccgtgtctgtggccgctggcgacagcaccgtgctgaactgtaccctgaccagcctgctgcccgtgggccccatcagatggtatagaggcgtgggccctagcagactgctgatctacagcttcgctggcgagtacgtgcccagaatcagaaacgtgtccgacaccaccaagcggaacaacatggacttcagcatcaggatcagcaacgtgacccctgccgacgccggcatctactactgcgtgaagttccagaagggcagcagcgagcccgacaccgagattcagtctggcggcggaaccgaggtgtacgtgctggctaagcccagccctcctgaggtgtccggccctgctgatagaggcatccccgaccagaaagtgaacttcacatgcaagagccacggcttcagccccagaaacatcaccctgaagtggttcaaggacggccaggaactgcaccccctggaaaccaccgtgaaccccagcggcaagaacgtgtcctacaacatcagctccaccgtgcgggtggtgctgaacagcatggacgtgaacagcaaagtgatctgcgaggtggcccacatcacactggacagaagccccctgagaggaatcgccaacctgagcaacttcatcagagtgtccccaaccgtgaaagtgacacagcagagccccaccagcatgaaccaagtgaacctgacctgcagagccgagagattctaccccgaggacctgcagctgatctggctggaaaacggcaacgtgtccagaaacgacacccccaagaacctgacaaagaacaccgacggcacctacaactacacctccctgtttctcgtgaactcctccgcccaccgcgaggacgtggtgttcacgtgccaagtgaagcacgaccagcagcccgccatcaccagaaaccacacagtgctgggcttcgcccacagcagcgaccagggcagcatgcagaccttccccgacaacaacgccacccacaactggaactgccacacccagagcagccccaagctgttctgggctctggtggtggtggccggcgtgctgttttgttacggcctgctcgtgaccgtggccctgtgcgtgatctggaccaacagcagaagaaacagaggcggccagagcgactacatgaacatgacccccagaaggcctggcctgacccggaagccttaccagccttacgcccctgccagagacttcgccgcctacagacct

SEQ ID NO: 57 - DNA, 1332 bp, Artificial Sequence
  muSIRP alpha -6aas-CD28cys
atggaacctgctggacctgcccctggcagactgggacctctgctgctgtgcctgctgctgagcgccagctgtttctgtaccggcgccaccggcaaagaactgaaagtgacccagcccgagaagtccgtgtctgtggccgctggcgacagcaccgtgctgaactgtaccctgaccagcctgctgcccgtgggccccatcagatggtatagaggcgtgggccctagcagactgctgatctacagcttcgctggcgagtacgtgcccagaatcagaaacgtgtccgacaccaccaagcggaacaacatggacttcagcatcaggatcagcaacgtgacccctgccgacgccggcatctactactgcgtgaagttccagaagggcagcagcgagcccgacaccgagattcagtctggcggcggaaccgaggtgtacgtgctggctaagcccagccctcctgaggtgtccggccctgctgatagaggcatccccgaccagaaagtgaacttcacatgcaagagccacggcttcagccccagaaacatcaccctgaagtggttcaaggacggccaggaactgcaccccctggaaaccaccgtgaaccccagcggcaagaacgtgtcctacaacatcagctccaccgtgcgggtggtgctgaacagcatggacgtgaacagcaaagtgatctgcgaggtggcccacatcacactggacagaagccccctgagaggaatcgccaacctgagcaacttcatcagagtgtccccaaccgtgaaagtgacacagcagagccccaccagcatgaaccaagtgaacctgacctgcagagccgagagattctaccccgaggacctgcagctgatctggctggaaaacggcaacgtgtccagaaacgacacccccaagaacctgacaaagaacaccgacggcacctacaactacacctccctgtttctcgtgaactcctccgcccaccgcgaggacgtggtgttcacgtgccaagtgaagcacgaccagcagcccgccatcaccagaaaccacacagtgctgggcttcgcccacagcagcgaccagggcagcatgcagaccttccccgacaacaactgccacacccagagcagccccaagctgttctgggctctggtggtggtggccggcgtgctgttttgttacggcctgctcgtgaccgtggccctgtgcgtgatctggaccaacagcagaagaaacagaggcggccagagcgactacatgaacatgacccccagaaggcctggcctgacccggaagccttaccagccttacgcccctgccagagacttcgccgcctacagacct

SEQ ID NO: 58 - DNA, 1323 bp, Artificial Sequence
  muSIRP alpha -9aas-CD28cys
atggaacctgctggacctgcccctggcagactgggacctctgctgctgtgcctgctgctgagcgccagctgtttctgtaccggcgccaccggcaaagaactgaaagtgacccagcccgagaagtccgtgtctgtggccgctggcgacagcaccgtgctgaactgtaccctgaccagcctgctgcccgtgggccccatcagatggtatagaggcgtgggccctagcagactgctgatctacagcttcgctggcgagtacgtgcccagaatcagaaacgtgtccgacaccaccaagcggaacaacatggacttcagcatcaggatcagcaacgtgacccctgccgacgccggcatctactactgcgtgaagttccagaagggcagcagcgagcccgacaccgagattcagtctggcggcggaaccgaggtgtacgtgctggctaagcccagccctcctgaggtgtccggccctgctgatagaggcatccccgaccagaaagtgaacttcacatgcaagagccacggcttcagccccagaaacatcaccctgaagtggttcaaggacggccaggaactgcaccccctggaaaccaccgtgaaccccagcggcaagaacgtgtcctacaacatcagctccaccgtgcgggtggtgctgaacagcatggacgtgaacagcaaagtgatctgcgaggtggcccacatcacactggacagaagccccctgagaggaatcgccaacctgagcaacttcatcagagtgtccccaaccgtgaaagtgacacagcagagccccaccagcatgaaccaagtgaacctgacctgcagagccgagagattctaccccgaggacctgcagctgatctggctggaaaacggcaacgtgtccagaaacgacacccccaagaacctgacaaagaacaccgacggcacctacaactacacctccctgtttctcgtgaactcctccgcccaccgcgaggacgtggtgttcacgtgccaagtgaagcacgaccagcagcccgccatcaccagaaaccacacagtgctgggcttcgcccacagcagcgaccagggcagcatgcagaccttcccctgccacacccagagcagccccaagctgttctgggctctggtggtggtggccggcgtgctgttttgttacggcctgctcgtgaccgtggccctgtgcgtgatctggaccaacagcagaagaaacagaggcggccagagcgactacatgaacatgacccccagaaggcctggcctgacccggaagccttaccagccttacgcccctgccagagacttcgccgcctacagacct

SEQ ID NO: 59 - DNA, 1281 bp, Artificial Sequence
  muSIRP alpha-23aas-CD28cys
atggaacctgctggacctgcccctggcagactgggacctctgctgctgtgcctgctgctgagcgccagctgtttctgtaccggcgccaccggcaaagaactgaaagtgacccagcccgagaagtccgtgtctgtggccgctggcgacagcaccgtgctgaactgtaccctgaccagcctgctgcccgtgggccccatcagatggtatagaggcgtgggccctagcagactgctgatctacagcttcgctggcgagtacgtgcccagaatcagaaacgtgtccgacaccaccaagcggaacaacatggacttcagcatcaggatcagcaacgtgacccctgccgacgccggcatctactactgcgtgaagttccagaagggcagcagcgagcccgacaccgagattcagtctggcggcggaaccgaggtgtacgtgctggctaagcccagccctcctgaggtgtccggccctgctgatagaggcatccccgaccagaaagtgaacttcacatgcaagagccacggcttcagccccagaaacatcaccctgaagtggttcaaggacggccaggaactgcaccccctggaaaccaccgtgaaccccagcggcaagaacgtgtcctacaacatcagctccaccgtgcgggtggtgctgaacagcatggacgtgaacagcaaagtgatctgcgaggtggcccacatcacactggacagaagccccctgagaggaatcgccaacctgagcaacttcatcagagtgtccccaaccgtgaaagtgacacagcagagccccaccagcatgaaccaagtgaacctgacctgcagagccgagagattctaccccgaggacctgcagctgatctggctggaaaacggcaacgtgtccagaaacgacacccccaagaacctgacaaagaacaccgacggcacctacaactacacctccctgtttctcgtgaactcctccgcccaccgcgaggacgtggtgttcacgtgccaagtgaagcacgaccagcagcccgccatcaccagaaaccacacagtgctgggctgccacacccagagcagccccaagctgttctgggctctggtggtggtggccggcgtgctgttttgttacggcctgctcgtgaccgtggccctgtgcgtgatctggaccaacagcagaagaaacagaggcggccagagcgactacatgaacatgacccccagaaggcctggcctgacccggaagccttaccagccttacgcccctgccagagacttcgccgcctacagacct

SEQ ID NO: 60 - protein, 137 aa, Artificial Sequence
  huPD-1 ectodomain
PPTFSPALLVVTEGDNATFTCSFSNTSESFVLNWYRMSPSNQTDKLAAFPEDRSQPGQDCRFRVTQLPNGRDFHMSVVRARRNDSGTYLCGAISLAPKAQIKESLRAELRVTERRAEVPTAHPSPSPRSAGQFQTLV

SEQ ID NO: 61 - DNA, 627 bp, Artificial Sequence
  huCD2 entire extracellular domain
atgagctttccatgtaaatttgtagccagcttccttctgattttcaatgtttcttccaaaggtgcagtctccaaagagattacgaatgccttggaaacctggggtgccttgggtcaggacatcaacttggacattcctagttttcaaatgagtgatgatattgacgatataaaatgggaaaaaacttcagacaagaaaaagattgcacaattcagaaaagagaaagagactttcaaggaaaaagatacatataagctatttaaaaatggaactctgaaaattaagcatctgaagaccgatgatcaggatatctacaaggtatcaatatatgatacaaaaggaaaaaatgtgttggaaaaaatatttgatttgaagattcaagagagggtctcaaaaccaaagatctcctggacttgtatcaacacaaccctgacctgtgaggtaatgaatggaactgaccccgaattaaacctgtatcaagatgggaaacatctaaaactttctcagagggtcatcacacacaagtggaccaccagcctgagtgcaaaattcaagtgcacagcagggaacaaagtcagcaaggaatccagtgtcgagcctgtcagctgtccagagaaaggtctggac

SEQ ID NO: 62 - protein, 209 aa, Artificial Sequence
  huCD2 entire extracellular domain
MSFPCKFVASFLLIFNVSSKGAVSKEITNALETWGALGQDINLDIPSFQMSDDIDDIKWEKTSDKKKIAQFRKEKETFKEKDTYKLFKNGTLKIKHLKTDDQDIYKVSIYDTKGKNVLEKIFDLKIQERVSKPKISWTCINTTLTCEVMNGTDPELNLYQDGKHLKLSQRVITHKWTTSLSAKFKCTAGNKVSKESSVEPVSCPEKGLD

SEQ ID NO: 63 - DNA, 78 bp, Artificial Sequence
  huCD2 transmembrane domain
atctatctcatcattggcatatgtggaggaggcagcctcttgatggtctttgtggcactgctcgttttctatatcacc

SEQ ID NO: 64 - protein, 26 aa, Artificial Sequence
  huCD2 transmembrane domain
IYLIIGICGGGSLLMVFVALLVFYIT

SEQ ID NO: 65 - DNA, 828 bp, Artificial Sequence
  huCD2tm-CD28 DNA
atgagctttccatgtaaatttgtagccagcttccttctgattttcaatgtttcttccaaaggtgcagtctccaaagagattacgaatgccttggaaacctggggtgccttgggtcaggacatcaacttggacattcctagttttcaaatgagtgatgatattgacgatataaaatgggaaaaaacttcagacaagaaaaagattgcacaattcagaaaagagaaagagactttcaaggaaaaagatacatataagctatttaaaaatggaactctgaaaattaagcatctgaagaccgatgatcaggatatctacaaggtatcaatatatgatacaaaaggaaaaaatgtgttggaaaaaatatttgatttgaagattcaagagagggtctcaaaaccaaagatctcctggacttgtatcaacacaaccctgacctgtgaggtaatgaatggaactgaccccgaattaaacctgtatcaagatgggaaacatctaaaactttctcagagggtcatcacacacaagtggaccaccagcctgagtgcaaaattcaagtgcacagcagggaacaaagtcagcaaggaatccagtgtcgagcctgtcagctgtccagagaaaggtctggacatctatctcatcattggcatatgtggaggaggcagcctcttgatggtctttgtggcactgctcgttttctatatcacccgcagcaagcggagcagaggcggccacagcgactacatgaacatgacccctagacggcctggccccaccagaaagcactaccagccctacgcccctccccgggactttgccgcctacagaagc

SEQ ID NO: 66 - protein, 276 aa, Artificial Sequence
  huCD2tm-CD28
MSFPCKFVASFLLIFNVSSKGAVSKEITNALETWGALGQDINLDIPSFQMSDDIDDIKWEKTSDKKKIAQFRKEKETFKEKDTYKLFKNGTLKIKHLKTDDQDIYKVSIYDTKGKNVLEKIFDLKIQERVSKPKISWTCINTTLTCEVMNGTDPELNLYQDGKHLKLSQRVITHKWTTSLSAKFKCTAGNKVSKESSVEPVSCPEKGLDIYLIIGICGGGSLLMVFVALLVFYITRSKRSRGGHSDYMNMTPRRPGPTRKHYQPYAPPRDFAAYRS

SEQ ID NO: 67 - DNA, 831 bp, Artificial Sequence
  huCD2-CD28tm
atgagctttccatgtaaatttgtagccagcttccttctgattttcaatgtttcttccaaaggtgcagtctccaaagagattacgaatgccttggaaacctggggtgccttgggtcaggacatcaacttggacattcctagttttcaaatgagtgatgatattgacgatataaaatgggaaaaaacttcagacaagaaaaagattgcacaattcagaaaagagaaagagactttcaaggaaaaagatacatataagctatttaaaaatggaactctgaaaattaagcatctgaagaccgatgatcaggatatctacaaggtatcaatatatgatacaaaaggaaaaaatgtgttggaaaaaatatttgatttgaagattcaagagagggtctcaaaaccaaagatctcctggacttgtatcaacacaaccctgacctgtgaggtaatgaatggaactgaccccgaattaaacctgtatcaagatgggaaacatctaaaactttctcagagggtcatcacacacaagtggaccaccagcctgagtgcaaaattcaagtgcacagcagggaacaaagtcagcaaggaatccagtgtcgagcctgtcagctgtccagagaaaggtctggacttctgggtgctggtggtggtcggaggcgtgctggcctgctacagcctgctggtcaccgtggccttcatcatcttttgggtccgcagcaagcggagcagaggcggccacagcgactacatgaacatgacccctagacggcctggccccaccagaaagcactaccagccctacgcccctccccgggactttgccgcctacagaagc

SEQ ID NO: 68 - protein, 277 aa, Artificial Sequence
  huCD2-CD28tm
MSFPCKFVASFLLIFNVSSKGAVSKEITNALETWGALGQDINLDIPSFQMSDDIDDIKWEKTSDKKKIAQFRKEKETFKEKDTYKLFKNGTLKIKHLKTDDQDIYKVSIYDTKGKNVLEKIFDLKIQERVSKPKISWTCINTTLTCEVMNGTDPELNLYQDGKHLKLSQRVITHKWTTSLSAKFKCTAGNKVSKESSVEPVSCPEKGLDFWVLVVVGGVLACYSLLVTVAFIIFWVRSKRSRGGHSDYMNMTPRRPGPTRKHYQPYAPPRDFAAYRS

SEQ ID NO: 69 - DNA, 969 bp, Artificial Sequence
  huCD200R-CD28Cys
atgctgtgcccttggagaaccgccaacctgggcctgctgctgatcctgaccatcttcctggtggccgccagcagcagcctgtgcatggacgagaagcagatcacccagaactacagcaaggtgctggccgaagtgaacaccagctggcccgtgaagatggccaccaacgccgtgctgtgctgccctcctatcgccctgcggaacctgatcatcatcacctgggagatcatcctgcggggccagcccagctgtaccaaggcctaccggaaagagacaaacgagacaaaagaaacaaactgcaccgacgagcggatcacatgggtgtccagacccgaccagaacagcgacctgcagatcagacccgtggccatcacccacgacggctactaccggtgcatcatggtcacccccgatggcaacttccaccggggataccatctgcaggtgctcgtgacccccgaagtgaccctgttccagaaccggaacagaaccgccgtgtgcaaggccgtggccggaaaacctgccgcccagatctcttggatccccgagggcgattgcgccaccaagcaggaatactggtccaacggcaccgtgaccgtgaagtccacctgtcactgggaggtgcacaacgtgtccaccgtgacatgccacgtgtcccacctgaccggcaacaagagcctgtacatcgagctgctgcctgtgcctggcgccaagaagtccgccaagctgtgtcccagccctctgtttcccggccctagcaagcctttctgggtgctggtggtggtcggaggcgtgctggcctgctacagcctgctggtcaccgtggccttcatcatcttttgggtccgcagcaagcggagcagaggcggccacagcgactacatgaacatgacccctagacggcctggccccaccagaaagcactaccagccctacgcccctccccgggactttgccgcctacagaagc

SEQ ID NO: 70 - protein, 323 aa, Artificial Sequence
  huCD200R-CD28Cys
MLCPWRTANLGLLLILTIFLVAASSSLCMDEKQITQNYSKVLAEVNTSWPVKMATNAVLCCPPIALRNLIIITWEIILRGQPSCTKAYRKETNETKETNCTDERITWVSRPDQNSDLQIRPVAITHDGYYRCIMVTPDGNFHRGYHLQVLVTPEVTLFQNRNRTAVCKAVAGKPAAQISWIPEGDCATKQEYWSNGTVTVKSTCHWEVHNVSTVTCHVSHLTGNKSLYIELLPVPGAKKSAKLCPSPLFPGPSKPFWVLVVVGGVLACYSLLVTVAFIIFWVRSKRSRGGHSDYMNMTPRRPGPTRKHYQPYAPPRDFAAYRS

SEQ ID NO: 71 - DNA, 519 bp, Artificial Sequence
  huFas entire extracellular domain
atgctgggcatctggaccctgctgcctctggtgctgacaagcgtggccagactgagcagcaagagcgtgaacgcccaagtgaccgacatcaacagcaagggcctggaactgagaaagaccgtgaccaccgtggaaacccagaacctggaaggcctgcaccacgacggccagttctgccacaagccttgtccccctggcgagcggaaggccagagactgtactgtgaacggcgacgagcccgactgcgtgccctgtcaggaaggcaaagagtacaccgacaaggcccacttcagcagcaagtgccggcggtgcagactgtgtgatgagggccacggcctggaagtggaaatcaactgcacccggacccagaacaccaagtgcagatgcaagcccaacttcttctgcaacagcaccgtgtgcgagcactgcgacccctgtaccaagtgcgaacacggcatcatcaaagagtgcaccctgacctccaacacaaagtgcaaagaggaaggcagcagaagcaac

SEQ ID NO: 72 - protein, 173 aa, Artificial Sequence
  huFas entire extracellular domain
MLGIWTLLPLVLTSVARLSSKSVNAQVTDINSKGLELRKTVTTVETQNLEGLHHDGQFCHKPCPPGERKARDCTVNGDEPDCVPCQEGKEYTDKAHFSSKCRRCRLCDEGHGLEVEINCTRTQNTKCRCKPNFFCNSTVCEHCDPCTKCEHGIIKECTLTSNTKCKEEGSRSN

SEQ ID NO: 73 - DNA, 498 bp, Artificial Sequence
  huFas extracellular domain -7aas
atgctgggcatctggaccctgctgcctctggtgctgacaagcgtggccagactgagcagcaagagcgtgaacgcccaagtgaccgacatcaacagcaagggcctggaactgagaaagaccgtgaccaccgtggaaacccagaacctggaaggcctgcaccacgacggccagttctgccacaagccttgtccccctggcgagcggaaggccagagactgtactgtgaacggcgacgagcccgactgcgtgccctgtcaggaaggcaaagagtacaccgacaaggcccacttcagcagcaagtgccggcggtgcagactgtgtgatgagggccacggcctggaagtggaaatcaactgcacccggacccagaacaccaagtgcagatgcaagcccaacttcttctgcaacagcaccgtgtgcgagcactgcgacccctgtaccaagtgcgaacacggcatcatcaaagagtgcaccctgacctccaacacaaagtgcaaa

SEQ ID NO: 74 - protein, 166 aa, Artificial Sequence
  huFas extracellular domain -7aas
MLGIWTLLPLVLTSVARLSSKSVNAQVTDINSKGLELRKTVTTVETQNLEGLHHDGQFCHKPCPPGERKARDCTVNGDEPDCVPCQEGKEYTDKAHFSSKCRRCRLCDEGHGLEVEINCTRTQNTKCRCKPNFFCNSTVCEHCDPCTKCEHGIIKECTLTSNTKCK

SEQ ID NO: 75 - DNA, 483 bp, Artificial Sequence
  huFas extracellular domain -12aas
atgctgggcatctggaccctgctgcctctggtgctgacaagcgtggccagactgagcagcaagagcgtgaacgcccaagtgaccgacatcaacagcaagggcctggaactgagaaagaccgtgaccaccgtggaaacccagaacctggaaggcctgcaccacgacggccagttctgccacaagccttgtccccctggcgagcggaaggccagagactgtactgtgaacggcgacgagcccgactgcgtgccctgtcaggaaggcaaagagtacaccgacaaggcccacttcagcagcaagtgccggcggtgcagactgtgtgatgagggccacggcctggaagtggaaatcaactgcacccggacccagaacaccaagtgcagatgcaagcccaacttcttctgcaacagcaccgtgtgcgagcactgcgacccctgtaccaagtgcgaacacggcatcatcaaagagtgcaccctgacctcc

SEQ ID NO: 76 - protein, 161 aa, Artificial Sequence
  huFas extracellular domain -12aas
MLGIWTLLPLVLTSVARLSSKSVNAQVTDINSKGLELRKTVTTVETQNLEGLHHDGQFCHKPCPPGERKARDCTVNGDEPDCVPCQEGKEYTDKAHFSSKCRRCRLCDEGHGLEVEINCTRTQNTKCRCKPNFFCNSTVCEHCDPCTKCEHGIIKECTLTS

SEQ ID NO: 77 - DNA, 51 bp, Artificial Sequence
  huFas transmembrane domain
ctgggctggctgtgcctcctgctgctgcccatccctctgatcgtgtgggtc

SEQ ID NO: 78 - protein, 17 aa, Artificial Sequence
  huFas transmembrane domain
LGWLCLLLLPIPLIVWV

SEQ ID NO: 79 - DNA, 693 bp, Artificial Sequence
  huFAStm-CD28
atgctgggcatctggaccctgctgcctctggtgctgacaagcgtggccagactgagcagcaagagcgtgaacgcccaagtgaccgacatcaacagcaagggcctggaactgagaaagaccgtgaccaccgtggaaacccagaacctggaaggcctgcaccacgacggccagttctgccacaagccttgtccccctggcgagcggaaggccagagactgtactgtgaacggcgacgagcccgactgcgtgccctgtcaggaaggcaaagagtacaccgacaaggcccacttcagcagcaagtgccggcggtgcagactgtgtgatgagggccacggcctggaagtggaaatcaactgcacccggacccagaacaccaagtgcagatgcaagcccaacttcttctgcaacagcaccgtgtgcgagcactgcgacccctgtaccaagtgcgaacacggcatcatcaaagagtgcaccctgacctccaacacaaagtgcaaagaggaaggcagcagaagcaacctgggctggctgtgcctcctgctgctgcccatccctctgatcgtgtgggtccgcagcaagcggagcagaggcggccacagcgactacatgaacatgacccctagacggcctggccccaccagaaagcactaccagccctacgcccctccccgggactttgccgcctacagaagc

SEQ ID NO: 80 - protein, 231 aa, Artificial Sequence
  huFAStm-CD28
MLGIWTLLPLVLTSVARLSSKSVNAQVTDINSKGLELRKTVTTVETQNLEGLHHDGQFCHKPCPPGERKARDCTVNGDEPDCVPCQEGKEYTDKAHFSSKCRRCRLCDEGHGLEVEINCTRTQNTKCRCKPNFFCNSTVCEHCDPCTKCEHGIIKECTLTSNTKCKEEGSRSNLGWLCLLLLPIPLIVWVRSKRSRGGHSDYMNMTPRRPGPTRKHYQPYAPPRDFAAYRS

SEQ ID NO: 81 - DNA, 723 bp, Artificial Sequence
  huFAS-CD28tm
atgctgggcatctggaccctgctgcctctggtgctgacaagcgtggccagactgagcagcaagagcgtgaacgcccaagtgaccgacatcaacagcaagggcctggaactgagaaagaccgtgaccaccgtggaaacccagaacctggaaggcctgcaccacgacggccagttctgccacaagccttgtccccctggcgagcggaaggccagagactgtactgtgaacggcgacgagcccgactgcgtgccctgtcaggaaggcaaagagtacaccgacaaggcccacttcagcagcaagtgccggcggtgcagactgtgtgatgagggccacggcctggaagtggaaatcaactgcacccggacccagaacaccaagtgcagatgcaagcccaacttcttctgcaacagcaccgtgtgcgagcactgcgacccctgtaccaagtgcgaacacggcatcatcaaagagtgcaccctgacctccaacacaaagtgcaaagaggaaggcagcagaagcaacttctgggtgctggtggtggtcggaggcgtgctggcctgctacagcctgctggtcaccgtggccttcatcatcttttgggtccgcagcaagcggagcagaggcggccacagcgactacatgaacatgacccctagacggcctggccccaccagaaagcactaccagccctacgcccctccccgggactttgccgcctacagaagc

SEQ ID NO: 82 - protein, 241 aa, Artificial Sequence
  huFAS-CD28tm
MLGIWTLLPLVLTSVARLSSKSVNAQVTDINSKGLELRKTVTTVETQNLEGLHHDGQFCHKPCPPGERKARDCTVNGDEPDCVPCQEGKEYTDKAHFSSKCRRCRLCDEGHGLEVEINCTRTQNTKCRCKPNFFCNSTVCEHCDPCTKCEHGIIKECTLTSNTKCKEEGSRSNFWVLVVVGGVLACYSLLVTVAFIIFWVRSKRSRGGHSDYMNMTPRRPGPTRKHYQPYAPPRDFAAYRS

SEQ ID NO: 83 - DNA, 759 bp, Artificial Sequence
  huFAS-CD28Cys
atgctgggcatctggaccctgctgcctctggtgctgacaagcgtggccagactgagcagcaagagcgtgaacgcccaagtgaccgacatcaacagcaagggcctggaactgagaaagaccgtgaccaccgtggaaacccagaacctggaaggcctgcaccacgacggccagttctgccacaagccttgtccccctggcgagcggaaggccagagactgtactgtgaacggcgacgagcccgactgcgtgccctgtcaggaaggcaaagagtacaccgacaaggcccacttcagcagcaagtgccggcggtgcagactgtgtgatgagggccacggcctggaagtggaaatcaactgcacccggacccagaacaccaagtgcagatgcaagcccaacttcttctgcaacagcaccgtgtgcgagcactgcgacccctgtaccaagtgcgaacacggcatcatcaaagagtgcaccctgacctccaacacaaagtgcaaagaggaaggcagcagaagcaactgtcccagccctctgtttcccggccctagcaagcctttctgggtgctggtggtggtcggaggcgtgctggcctgctacagcctgctggtcaccgtggccttcatcatcttttgggtccgcagcaagcggagcagaggcggccacagcgactacatgaacatgacccctagacggcctggccccaccagaaagcactaccagccctacgcccctccccgggactttgccgcctacagaagc

SEQ ID NO: 84 - protein, 253 aa, Artificial Sequence
  huFAS-CD28Cys
MLGIWTLLPLVLTSVARLSSKSVNAQVTDINSKGLELRKTVTTVETQNLEGLHHDGQFCHKPCPPGERKARDCTVNGDEPDCVPCQEGKEYTDKAHFSSKCRRCRLCDEGHGLEVEINCTRTQNTKCRCKPNFFCNSTVCEHCDPCTKCEHGIIKECTLTSNTKCKEEGSRSNCPSPLFPGPSKPFWVLVVVGGVLACYSLLVTVAFIIFWVRSKRSRGGHSDYMNMTPRRPGPTRKHYQPYAPPRDFAAYRS

SEQ ID NO: 85 - DNA, 738 bp, Artificial Sequence
  huFAS-7aas-CD28Cys
atgctgggcatctggaccctgctgcctctggtgctgacaagcgtggccagactgagcagcaagagcgtgaacgcccaagtgaccgacatcaacagcaagggcctggaactgagaaagaccgtgaccaccgtggaaacccagaacctggaaggcctgcaccacgacggccagttctgccacaagccttgtccccctggcgagcggaaggccagagactgtactgtgaacggcgacgagcccgactgcgtgccctgtcaggaaggcaaagagtacaccgacaaggcccacttcagcagcaagtgccggcggtgcagactgtgtgatgagggccacggcctggaagtggaaatcaactgcacccggacccagaacaccaagtgcagatgcaagcccaacttcttctgcaacagcaccgtgtgcgagcactgcgacccctgtaccaagtgcgaacacggcatcatcaaagagtgcaccctgacctccaacacaaagtgcaaatgtcccagccctctgtttcccggccctagcaagcctttctgggtgctggtggtggtcggaggcgtgctggcctgctacagcctgctggtcaccgtggccttcatcatcttttgggtccgcagcaagcggagcagaggcggccacagcgactacatgaacatgacccctagacggcctggccccaccagaaagcactaccagccctacgcccctccccgggactttgccgcctacagaagc

SEQ ID NO: 86 - protein, 246 aa, Artificial Sequence
  huFAS-7aas-CD28Cys
MLGIWTLLPLVLTSVARLSSKSVNAQVTDINSKGLELRKTVTTVETQNLEGLHHDGQFCHKPCPPGERKARDCTVNGDEPDCVPCQEGKEYTDKAHFSSKCRRCRLCDEGHGLEVEINCTRTQNTKCRCKPNFFCNSTVCEHCDPCTKCEHGIIKECTLTSNTKCKCPSPLFPGPSKPFWVLVVVGGVLACYSLLVTVAFIIFWVRSKRSRGGHSDYMNMTPRRPGPTRKHYQPYAPPRDFAAYRS

SEQ ID NO: 87 - DNA, 723 bp, Artificial Sequence
  FAS-12aas-CD28Cys
atgctgggcatctggaccctgctgcctctggtgctgacaagcgtggccagactgagcagcaagagcgtgaacgcccaagtgaccgacatcaacagcaagggcctggaactgagaaagaccgtgaccaccgtggaaacccagaacctggaaggcctgcaccacgacggccagttctgccacaagccttgtccccctggcgagcggaaggccagagactgtactgtgaacggcgacgagcccgactgcgtgccctgtcaggaaggcaaagagtacaccgacaaggcccacttcagcagcaagtgccggcggtgcagactgtgtgatgagggccacggcctggaagtggaaatcaactgcacccggacccagaacaccaagtgcagatgcaagcccaacttcttctgcaacagcaccgtgtgcgagcactgcgacccctgtaccaagtgcgaacacggcatcatcaaagagtgcaccctgacctcctgtcccagccctctgtttcccggccctagcaagcctttctgggtgctggtggtggtcggaggcgtgctggcctgctacagcctgctggtcaccgtggccttcatcatcttttgggtccgcagcaagcggagcagaggcggccacagcgactacatgaacatgacccctagacggcctggccccaccagaaagcactaccagccctacgcccctccccgggactttgccgcctacagaagc

SEQ ID NO: 88 - protein, 241 aa, Artificial Sequence
  FAS-12aas-CD28Cys
MLGIWTLLPLVLTSVARLSSKSVNAQVTDINSKGLELRKTVTTVETQNLEGLHHDGQFCHKPCPPGERKARDCTVNGDEPDCVPCQEGKEYTDKAHFSSKCRRCRLCDEGHGLEVEINCTRTQNTKCRCKPNFFCNSTVCEHCDPCTKCEHGIIKECTLTSCPSPLFPGPSKPFWVLVVVGGVLACYSLLVTVAFIIFWVRSKRSRGGHSDYMNMTPRRPGPTRKHYQPYAPPRDFAAYRS

SEQ ID NO: 89 - DNA, 510 bp, Artificial Sequence
  huPD1 entire extracellular domain 2
atgcagatccctcaggccccttggcctgtcgtgtgggctgtgctgcagctgggatggcggcctggctggtttctggacagccccgacagaccctggaacccccctacattttcccctgccctgctggtcgtgaccgagggcgacaatgccaccttcacctgtagcttcagcaacaccagcgagagcttcgtgctgaactggtacagaatgagccccagcaaccagaccgacaagctggccgccttccccgaggatagatctcagcccggccaggactgccggttcagagtgacccagctgcccaacggccgggacttccacatgtctgtcgtgcgggccagacggaacgacagcggcacatatctgtgcggcgccatcagcctggcccccaaggcccagatcaaagagagcctgagagccgagctgagagtgaccgagagaagggccgaagtgcctaccgcccaccctagcccatctccaagacctgccggccagttccagacactggtc

SEQ ID NO: 90 - protein, 170 aa, Artificial Sequence
  huPD1 entire extracellular domain 2
MQIPQAPWPVVWAVLQLGWRPGWFLDSPDRPWNPPTFSPALLVVTEGDNATFTCSFSNTSESFVLNWYRMSPSNQTDKLAAFPEDRSQPGQDCRFRVTQLPNGRDFHMSVVRARRNDSGTYLCGAISLAPKAQIKESLRAELRVTERRAEVPTAHPSPSPRPAGQFQTLV

SEQ ID NO: 91 - DNA, 474 bp, Artificial Sequence
  huPD1 2 -12aas
atgcagatccctcaggccccttggcctgtcgtgtgggctgtgctgcagctgggatggcggcctggctggtttctggacagccccgacagaccctggaacccccctacattttcccctgccctgctggtcgtgaccgagggcgacaatgccaccttcacctgtagcttcagcaacaccagcgagagcttcgtgctgaactggtacagaatgagccccagcaaccagaccgacaagctggccgccttccccgaggatagatctcagcccggccaggactgccggttcagagtgacccagctgcccaacggccgggacttccacatgtctgtcgtgcgggccagacggaacgacagcggcacatatctgtgcggcgccatcagcctggcccccaaggcccagatcaaagagagcctgagagccgagctgagagtgaccgagagaagggccgaagtgcctaccgcccaccctagccca

SEQ ID NO: 92 - protein, 158 aa, Artificial Sequence
  huPD1 2 -12aas
MQIPQAPWPVVWAVLQLGWRPGWFLDSPDRPWNPPTFSPALLVVTEGDNATFTCSFSNTSESFVLNWYRMSPSNQTDKLAAFPEDRSQPGQDCRFRVTQLPNGRDFHMSVVRARRNDSGTYLCGAISLAPKAQIKESLRAELRVTERRAEVPTAHPSP

SEQ ID NO: 93 - DNA, 465 bp, Artificial Sequence
  huPD1 2 -15aas
atgcagatccctcaggccccttggcctgtcgtgtgggctgtgctgcagctgggatggcggcctggctggtttctggacagccccgacagaccctggaacccccctacattttcccctgccctgctggtcgtgaccgagggcgacaatgccaccttcacctgtagcttcagcaacaccagcgagagcttcgtgctgaactggtacagaatgagccccagcaaccagaccgacaagctggccgccttccccgaggatagatctcagcccggccaggactgccggttcagagtgacccagctgcccaacggccgggacttccacatgtctgtcgtgcgggccagacggaacgacagcggcacatatctgtgcggcgccatcagcctggcccccaaggcccagatcaaagagagcctgagagccgagctgagagtgaccgagagaagggccgaagtgcctaccgcccac

SEQ ID NO: 94 - protein, 155 aa, Artificial Sequence
  huPD1 2 -15aas
MQIPQAPWPVVWAVLQLGWRPGWFLDSPDRPWNPPTFSPALLVVTEGDNATFTCSFSNTSESFVLNWYRMSPSNQTDKLAAFPEDRSQPGQDCRFRVTQLPNGRDFHMSVVRARRNDSGTYLCGAISLAPKAQIKESLRAELRVTERRAEVPTAH

SEQ ID NO: 95 - DNA, 447 bp, Artificial Sequence
  huPD1 2 -21aas
atgcagatccctcaggccccttggcctgtcgtgtgggctgtgctgcagctgggatggcggcctggctggtttctggacagccccgacagaccctggaacccccctacattttcccctgccctgctggtcgtgaccgagggcgacaatgccaccttcacctgtagcttcagcaacaccagcgagagcttcgtgctgaactggtacagaatgagccccagcaaccagaccgacaagctggccgccttccccgaggatagatctcagcccggccaggactgccggttcagagtgacccagctgcccaacggccgggacttccacatgtctgtcgtgcgggccagacggaacgacagcggcacatatctgtgcggcgccatcagcctggcccccaaggcccagatcaaagagagcctgagagccgagctgagagtgaccgagagaagggcc

SEQ ID NO: 96 - protein, 149 aa, Artificial Sequence
  huPD1 2 -21aas
MQIPQAPWPVVWAVLQLGWRPGWFLDSPDRPWNPPTFSPALLVVTEGDNATFTCSFSNTSESFVLNWYRMSPSNQTDKLAAFPEDRSQPGQDCRFRVTQLPNGRDFHMSVVRARRNDSGTYLCGAISLAPKAQIKESLRAELRVTERRA

SEQ ID NO: 97 - DNA, 750 bp, Artificial Sequence
  huPD1-CD28Cys
atgcagatccctcaggccccttggcctgtcgtgtgggctgtgctgcagctgggatggcggcctggctggtttctggacagccccgacagaccctggaacccccctacattttcccctgccctgctggtcgtgaccgagggcgacaatgccaccttcacctgtagcttcagcaacaccagcgagagcttcgtgctgaactggtacagaatgagccccagcaaccagaccgacaagctggccgccttccccgaggatagatctcagcccggccaggactgccggttcagagtgacccagctgcccaacggccgggacttccacatgtctgtcgtgcgggccagacggaacgacagcggcacatatctgtgcggcgccatcagcctggcccccaaggcccagatcaaagagagcctgagagccgagctgagagtgaccgagagaagggccgaagtgcctaccgcccaccctagcccatctccaagacctgccggccagttccagacactggtctgtcccagccctctgtttcccggccctagcaagcctttctgggtgctggtggtggtcggaggcgtgctggcctgctacagcctgctggtcaccgtggccttcatcatcttttgggtccgcagcaagcggagcagaggcggccacagcgactacatgaacatgacccctagacggcctggccccaccagaaagcactaccagccctacgcccctccccgggactttgccgcctacagaagc

SEQ ID NO: 98 - protein, 250 aa, Artificial Sequence
  huPD1-CD28Cys
MQIPQAPWPVVWAVLQLGWRPGWFLDSPDRPWNPPTFSPALLVVTEGDNATFTCSFSNTSESFVLNWYRMSPSNQTDKLAAFPEDRSQPGQDCRFRVTQLPNGRDFHMSVVRARRNDSGTYLCGAISLAPKAQIKESLRAELRVTERRAEVPTAHPSPSPRPAGQFQTLVCPSPLFPGPSKPFWVLVVVGGVLACYSLLVTVAFIIFWVRSKRSRGGHSDYMNMTPRRPGPTRKHYQPYAPPRDFAAYRS

SEQ ID NO: 99 - DNA, 714 bp, Artificial Sequence
  huPD1-12aas-CD28Cys
atgcagatccctcaggccccttggcctgtcgtgtgggctgtgctgcagctgggatggcggcctggctggtttctggacagccccgacagaccctggaacccccctacattttcccctgccctgctggtcgtgaccgagggcgacaatgccaccttcacctgtagcttcagcaacaccagcgagagcttcgtgctgaactggtacagaatgagccccagcaaccagaccgacaagctggccgccttccccgaggatagatctcagcccggccaggactgccggttcagagtgacccagctgcccaacggccgggacttccacatgtctgtcgtgcgggccagacggaacgacagcggcacatatctgtgcggcgccatcagcctggcccccaaggcccagatcaaagagagcctgagagccgagctgagagtgaccgagagaagggccgaagtgcctaccgcccaccctagcccatgtcccagccctctgtttcccggccctagcaagcctttctgggtgctggtggtggtcggaggcgtgctggcctgctacagcctgctggtcaccgtggccttcatcatcttttgggtccgcagcaagcggagcagaggcggccacagcgactacatgaacatgacccctagacggcctggccccaccagaaagcactaccagccctacgcccctccccgggactttgccgcctacagaagc

SEQ ID NO: 100 - protein, 238 aa, Artificial Sequence
  huPD1-12aas-CD28Cys
MQIPQAPWPVVWAVLQLGWRPGWFLDSPDRPWNPPTFSPALLVVTEGDNATFTCSFSNTSESFVLNWYRMSPSNQTDKLAAFPEDRSQPGQDCRFRVTQLPNGRDFHMSVVRARRNDSGTYLCGAISLAPKAQIKESLRAELRVTERRAEVPTAHPSPCPSPLFPGPSKPFWVLVVVGGVLACYSLLVTVAFIIFWVRSKRSRGGHSDYMNMTPRRPGPTRKHYQPYAPPRDFAAYRS

SEQ ID NO: 101 - DNA, 705 bp, Artificial Sequence
  huPD1-15aas-CD28Cys
atgcagatccctcaggccccttggcctgtcgtgtgggctgtgctgcagctgggatggcggcctggctggtttctggacagccccgacagaccctggaacccccctacattttcccctgccctgctggtcgtgaccgagggcgacaatgccaccttcacctgtagcttcagcaacaccagcgagagcttcgtgctgaactggtacagaatgagccccagcaaccagaccgacaagctggccgccttccccgaggatagatctcagcccggccaggactgccggttcagagtgacccagctgcccaacggccgggacttccacatgtctgtcgtgcgggccagacggaacgacagcggcacatatctgtgcggcgccatcagcctggcccccaaggcccagatcaaagagagcctgagagccgagctgagagtgaccgagagaagggccgaagtgcctaccgcccactgtcccagccctctgtttcccggccctagcaagcctttctgggtgctggtggtggtcggaggcgtgctggcctgctacagcctgctggtcaccgtggccttcatcatcttttgggtccgcagcaagcggagcagaggcggccacagcgactacatgaacatgacccctagacggcctggccccaccagaaagcactaccagccctacgcccctccccgggactttgccgcctacagaagc

SEQ ID NO: 102 - protein, 235 aa, Artificial Sequence
  huPD1-15aas-CD28Cys
MQIPQAPWPVVWAVLQLGWRPGWFLDSPDRPWNPPTFSPALLVVTEGDNATFTCSFSNTSESFVLNWYRMSPSNQTDKLAAFPEDRSQPGQDCRFRVTQLPNGRDFHMSVVRARRNDSGTYLCGAISLAPKAQIKESLRAELRVTERRAEVPTAHCPSPLFPGPSKPFWVLVVVGGVLACYSLLVTVAFIIFWVRSKRSRGGHSDYMNMTPRRPGPTRKHYQPYAPPRDFAAYRS

SEQ ID NO: 103 - DNA, 687 bp, Artificial Sequence
  huPD1-21aas-CD28Cys
atgcagatccctcaggccccttggcctgtcgtgtgggctgtgctgcagctgggatggcggcctggctggtttctggacagccccgacagaccctggaacccccctacattttcccctgccctgctggtcgtgaccgagggcgacaatgccaccttcacctgtagcttcagcaacaccagcgagagcttcgtgctgaactggtacagaatgagccccagcaaccagaccgacaagctggccgccttccccgaggatagatctcagcccggccaggactgccggttcagagtgacccagctgcccaacggccgggacttccacatgtctgtcgtgcgggccagacggaacgacagcggcacatatctgtgcggcgccatcagcctggcccccaaggcccagatcaaagagagcctgagagccgagctgagagtgaccgagagaagggcctgtcccagccctctgtttcccggccctagcaagcctttctgggtgctggtggtggtcggaggcgtgctggcctgctacagcctgctggtcaccgtggccttcatcatcttttgggtccgcagcaagcggagcagaggcggccacagcgactacatgaacatgacccctagacggcctggccccaccagaaagcactaccagccctacgcccctccccgggactttgccgcctacagaagc

SEQ ID NO: 104 - protein, 229 aa, Artificial Sequence
  huPD1-21aas-CD28Cys
MQIPQAPWPVVWAVLQLGWRPGWFLDSPDRPWNPPTFSPALLVVTEGDNATFTCSFSNTSESFVLNWYRMSPSNQTDKLAAFPEDRSQPGQDCRFRVTQLPNGRDFHMSVVRARRNDSGTYLCGAISLAPKAQIKESLRAELRVTERRACPSPLFPGPSKPFWVLVVVGGVLACYSLLVTVAFIIFWVRSKRSRGGHSDYMNMTPRRPGPTRKHYQPYAPPRDFAAYRS

SEQ ID NO: 105 - DNA, 810 bp, Artificial Sequence
  muCD2tm-CD28
atgaagtgcaagttcctgggctcattcttcctgctgttcagcctgagcggcaagggcgccgactgcagagacaacgagacaatctggggcgtgctgggccacggcatcaccctgaacatccccaacttccagatgaccgacgacatcgacgaagtgcgctgggtgcgaagaggcacactggtggccgagttcaagagaaagaagcccccattcctgatcagcgagacatacgaggtgctggccaacggcagcctgaagatcaagaaacccatgatgagaaacgacagcggcacctacaacgtgatggtgtacggcaccaacggcatgaccagactggaaaaggacctggacgtgcggatcctggaaagggtgtccaagcccatgatccactgggagtgccccaacaccaccctgacctgtgctgtgctgcagggcaccgacttcgagctgaagctgtaccagggcgagacactgctgaactccctgccccagaaaaacatgagctaccagtggaccaacctgaacgcccccttcaagtgcgaggccatcaaccccgtgtccaaagaaagcaagatggaagtcgtgaactgccccgagaagggcctgagcttctacgtgacagtgggcgtgggagctggcggactgctgctggtgctgctggtggccctgttcatcttctgcatctgcaacagcagacggaacagaggcggccagagcgactacatgaacatgacccccagaaggcctggcctgaccagaaagccctaccagccttacgcccctgccagagacttcgccgcctacagacct

SEQ ID NO: 106 - protein, 270 aa, Artificial Sequence
  muCD2tm-CD28
MKCKFLGSFFLLFSLSGKGADCRDNETIWGVLGHGITLNIPNFQMTDDIDEVRWVRRGTLVAEFKRKKPPFLISETYEVLANGSLKIKKPMMRNDSGTYNVMVYGTNGMTRLEKDLDVRILERVSKPMIHWECPNTTLTCAVLQGTDFELKLYQGETLLNSLPQKNMSYQWTNLNAPFKCEAINPVSKESKMEVVNCPEKGLSFYVTVGVGAGGLLLVLLVALFIFCICNSRRNRGGQSDYMNMTPRRPGLTRKPYQPYAPARDFAAYRP

SEQ ID NO: 107 - DNA, 813 bp, Artificial Sequence
  muCD2-CD28tm
atgaagtgcaagttcctgggctcattcttcctgctgttcagcctgagcggcaagggcgccgactgcagagacaacgagacaatctggggcgtgctgggccacggcatcaccctgaacatccccaacttccagatgaccgacgacatcgacgaagtgcgctgggtgcgaagaggcacactggtggccgagttcaagagaaagaagcccccattcctgatcagcgagacatacgaggtgctggccaacggcagcctgaagatcaagaaacccatgatgagaaacgacagcggcacctacaacgtgatggtgtacggcaccaacggcatgaccagactggaaaaggacctggacgtgcggatcctggaaagggtgtccaagcccatgatccactgggagtgccccaacaccaccctgacctgtgctgtgctgcagggcaccgacttcgagctgaagctgtaccagggcgagacactgctgaactccctgccccagaaaaacatgagctaccagtggaccaacctgaacgcccccttcaagtgcgaggccatcaaccccgtgtccaaagaaagcaagatggaagtcgtgaactgccccgagaagggcctgagcttctgggccctggtggtggtggccggcgtgctgttttgttacggcctgctcgtgaccgtggccctgtgcgtgatctggaccaacagcagaagaaacagaggcggccagagcgactacatgaacatgacccccagaaggcctggcctgaccagaaagccctaccagccttacgcccctgccagagacttcgccgcctacagaccc

SEQ ID NO: 108 - protein, 271 aa, Artificial Sequence
  muCD2-CD28tm
MKCKFLGSFFLLFSLSGKGADCRDNETIWGVLGHGITLNIPNFQMTDDIDEVRWVRRGTLVAEFKRKKPPFLISETYEVLANGSLKIKKPMMRNDSGTYNVMVYGTNGMTRLEKDLDVRILERVSKPMIHWECPNTTLTCAVLQGTDFELKLYQGETLLNSLPQKNMSYQWTNLNAPFKCEAINPVSKESKMEVVNCPEKGLSFWALVVVAGVLFCYGLLVTVALCVIWTNSRRNRGGQSDYMNMTPRRPGLTRKPYQPYAPARDFAAYRP

SEQ ID NO: 109 - DNA, 840 bp, Artificial Sequence
  muCD2-CD28Cys
atgaagtgcaagttcctgggctcattcttcctgctgttcagcctgagcggcaagggcgccgactgcagagacaacgagacaatctggggcgtgctgggccacggcatcaccctgaacatccccaacttccagatgaccgacgacatcgacgaagtgcgctgggtgcgaagaggcacactggtggccgagttcaagagaaagaagcccccattcctgatcagcgagacatacgaggtgctggccaacggcagcctgaagatcaagaaacccatgatgagaaacgacagcggcacctacaacgtgatggtgtacggcaccaacggcatgaccagactggaaaaggacctggacgtgcggatcctggaaagggtgtccaagcccatgatccactgggagtgccccaacaccaccctgacctgtgctgtgctgcagggcaccgacttcgagctgaagctgtaccagggcgagacactgctgaactccctgccccagaaaaacatgagctaccagtggaccaacctgaacgcccccttcaagtgcgaggccatcaaccccgtgtccaaagaaagcaagatggaagtcgtgaactgccccgagaagggcctgagctgccacacccagagcagccccaagctgttctgggccctggtggtggtggccggcgtgctgttttgttacggcctgctcgtgaccgtggccctgtgcgtgatctggaccaacagcagaagaaacagaggcggccagagcgactacatgaacatgacccccagaaggcctggcctgaccagaaagccctaccagccttacgcccctgccagagacttcgccgcctacagacct

SEQ ID NO: 110 - protein, 280 aa, Artificial Sequence
  muCD2-CD28Cys
MKCKFLGSFFLLFSLSGKGADCRDNETIWGVLGHGITLNIPNFQMTDDIDEVRWVRRGTLVAEFKRKKPPFLISETYEVLANGSLKIKKPMMRNDSGTYNVMVYGTNGMTRLEKDLDVRILERVSKPMIHWECPNTTLTCAVLQGTDFELKLYQGETLLNSLPQKNMSYQWTNLNAPFKCEAINPVSKESKMEVVNCPEKGLSCHTQSSPKLFWALVVVAGVLFCYGLLVTVALCVIWTNSRRNRGGQSDYMNMTPRRPGLTRKPYQPYAPARDFAAYRP

SEQ ID NO: 111 - DNA, 861 bp, Artificial Sequence
  muCD2-CD28Cys-41BBic
atgaagtgcaagttcctgggctcattcttcctgctgttcagcctgagcggcaagggcgccgactgcagagacaacgagacaatctggggcgtgctgggccacggcatcaccctgaacatccccaacttccagatgaccgacgacatcgacgaagtgcgctgggtgcgaagaggcacactggtggccgagttcaagagaaagaagcccccattcctgatcagcgagacatacgaggtgctggccaacggcagcctgaagatcaagaaacccatgatgagaaacgacagcggcacctacaacgtgatggtgtacggcaccaacggcatgaccagactggaaaaggacctggacgtgcggatcctggaaagggtgtccaagcccatgatccactgggagtgccccaacaccaccctgacctgtgctgtgctgcagggcaccgacttcgagctgaagctgtaccagggcgagacactgctgaactccctgccccagaaaaacatgagctaccagtggaccaacctgaacgcccccttcaagtgcgaggccatcaaccccgtgtccaaagaaagcaagatggaagtcgtgaactgccccgagaagggcctgagctgccacacccagagcagccccaagctgttctgggccctggtggtggtggccggcgtgctgttttgttacggcctgctcgtgaccgtggccctgtgcgtgatctggaccagcgtgctgaagtggatcagaaagaagttcccccacatcttcaagcagcccttcaagaaaaccaccggcgctgcccaggaagaggacgcctgcagctgtagatgccctcaggaagaagaaggcggcggaggcggctacgagctg

SEQ ID NO: 112 - protein, 287 aa, Artificial Sequence
  muCD2-CD28Cys-41BBic
MKCKFLGSFFLLFSLSGKGADCRDNETIWGVLGHGITLNIPNFQMTDDIDEVRWVRRGTLVAEFKRKKPPFLISETYEVLANGSLKIKKPMMRNDSGTYNVMVYGTNGMTRLEKDLDVRILERVSKPMIHWECPNTTLTCAVLQGTDFELKLYQGETLLNSLPQKNMSYQWTNLNAPFKCEAINPVSKESKMEVVNCPEKGLSCHTQSSPKLFWALVVVAGVLFCYGLLVTVALCVIWTSVLKWIRKKFPHIFKQPFKKTTGAAQEEDACSCRCPQEEEGGGGGYEL

SEQ ID NO: 113 - DNA, 1080 bp, Artificial Sequence
  muCD200R-3aas-CD28Cys tm ic-41BB
atgttctgcttctggcggacaagcgccctggccgtgctgctgatctggggagtgtttgtggccggcagcagctgcaccgacaagaaccagaccacccagaacaacagcagcagccccctgacccaagtgaacaccaccgtgtccgtgcagatcggcaccaaggccctgctgtgctgtttcagcatccctctgaccaaggctgtgctgatcacctggatcatcaagctgagaggcctgcccagctgcacaatcgcctacaaggtggacaccaagaccaacgagacaagctgcctgggcagaaacatcacctgggccagcaccccagaccacagccctgagctgcagatcagcgccgtgacactgcagcacgagggcacctacacatgcgagacagtgacccccgagggcaacttcgagaagaactacgatctgcaggtgctggtgccccccgaagtgacctacttccccgagaagaatagaagcgccgtgtgcgaggccatggctggcaaacctgccgcccagatctcttggagccctgacggcgactgtgtgaccaccagcgagagccacagcaacggcacagtgaccgtgcggagcacctgtcactgggagcagaacaacgtgtccgacgtgtcctgcatcgtgtcccacctgaccggcaaccagagcctgagcatcgagctgagcagaggcggaaaccagtcctgccacacccagagcagccccaagctgttctgggccctggtggtggtggccggcgtgctgttttgttacggcctgctcgtgaccgtggccctgtgcgtgatctggaccaacagcagaagaaacagaggcggccagagcgactacatgaacatgacccccagaaggcctggcctgaccagaaagccctaccagccttacgcccctgccagagacttcgccgcctacagacctagcgtgctgaagtggatcagaaagaagttcccccacatcttcaagcagcccttcaagaaaaccaccggcgctgcccaggaagaggacgcctgcagctgtagatgccctcaggaagaagaaggcggcggaggcggctacgagctg

SEQ ID NO: 114 - protein, 360 aa, Artificial Sequence
  muCD200R-3aas-CD28Cys tm ic-41BB
MFCFWRTSALAVLLIWGVFVAGSSCTDKNQTTQNNSSSPLTQVNTTVSVQIGTKALLCCFSIPLTKAVLITWIIKLRGLPSCTIAYKVDTKTNETSCLGRNITWASTPDHSPELQISAVTLQHEGTYTCETVTPEGNFEKNYDLQVLVPPEVTYFPEKNRSAVCEAMAGKPAAQISWSPDGDCVTTSESHSNGTVTVRSTCHWEQNNVSDVSCIVSHLTGNQSLSIELSRGGNQSCHTQSSPKLFWALVVVAGVLFCYGLLVTVALCVIWTNSRRNRGGQSDYMNMTPRRPGLTRKPYQPYAPARDFAAYRPSVLKWIRKKFPHIFKQPFKKTTGAAQEEDACSCRCPQEEEGGGGGYEL

SEQ ID NO: 115 - DNA, 966 bp, Artificial Sequence
  muCD200R-CD28Cys tm ic-41BB
atgttctgcttctggcggacaagcgccctggccgtgctgctgatctggggagtgtttgtggccggcagcagctgcaccgacaagaaccagaccacccagaacaacagcagcagccccctgacccaagtgaacaccaccgtgtccgtgcagatcggcaccaaggccctgctgtgctgtttcagcatccctctgaccaaggctgtgctgatcacctggatcatcaagctgagaggcctgcccagctgcacaatcgcctacaaggtggacaccaagaccaacgagacaagctgcctgggcagaaacatcacctgggccagcaccccagaccacagccctgagctgcagatcagcgccgtgacactgcagcacgagggcacctacacatgcgagacagtgacccccgagggcaacttcgagaagaactacgatctgcaggtgctggtgccccccgaagtgacctacttccccgagaagaatagaagcgccgtgtgcgaggccatggctggcaaacctgccgcccagatctcttggagccctgacggcgactgtgtgaccaccagcgagagccacagcaacggcacagtgaccgtgcggagcacctgtcactgggagcagaacaacgtgtccgacgtgtcctgcatcgtgtcccacctgaccggcaaccagagcctgagcatcgagctgagcagaggcggaaaccagtccctgaggccctgccacacccagagcagccccaagctgttctgggccctggtggtggtggccggcgtgctgttttgttacggcctgctcgtgaccgtggccctgtgcgtgatctggaccagcgtgctgaagtggatcagaaagaagttcccccacatcttcaagcagcccttcaagaaaaccaccggcgctgcccaggaagaggacgcctgcagctgtagatgccctcaggaagaagaaggcggcggaggcggctacgagctg

SEQ ID NO: 116 - protein, 322 aa, Artificial Sequence
  muCD200R-CD28Cys tm ic-41BB
MFCFWRTSALAVLLIWGVFVAGSSCTDKNQTTQNNSSSPLTQVNTTVSVQIGTKALLCCFSIPLTKAVLITWIIKLRGLPSCTIAYKVDTKTNETSCLGRNITWASTPDHSPELQISAVTLQHEGTYTCETVTPEGNFEKNYDLQVLVPPEVTYFPEKNRSAVCEAMAGKPAAQISWSPDGDCVTTSESHSNGTVTVRSTCHWEQNNVSDVSCIVSHLTGNQSLSIELSRGGNQSLRPCHTQSSPKLFWALVVVAGVLFCYGLLVTVALCVIWTSVLKWIRKKFPHIFKQPFKKTTGAAQEEDACSCRCPQEEEGGGGGYEL

SEQ ID NO: 117 - DNA, 681 bp, Artificial Sequence
  muFas tm-CD28
atgctgtggatctgggccgtgctgcctctggtgctggctggatcacagctgagagtgcacacccagggcaccaacagcatcagcgagagcctgaagctgagaagaagagtgcgcgagacagacaagaactgcagcgagggcctgtaccagggcggacccttctgctgtcagccttgccagcccggcaagaaaaaggtggaagattgcaagatgaacggcggcacccctacctgcgccccttgtacagagggcaaagagtacatggacaagaaccactacgccgacaagtgcagacggtgcaccctgtgcgacgaggaacacggcctggaagtggaaacaaactgcaccctgacccagaacaccaagtgcaagtgcaaacccgacttctactgcgacagccccggctgcgagcactgcgtcagatgtgcctcttgcgagcacggcaccctggaaccttgtaccgccaccagcaacaccaactgccggaagcagagccccagaaacagactgtggctgctgaccatcctggtgctgctgatccccctggtgttcatctacaacagcagaagaaacagaggcggccagagcgactacatgaacatgacccccagaaggcctggcctgaccagaaagccctaccagccttacgcccctgccagagacttcgccgcctacagacct

SEQ ID NO: 118 - protein, 227 aa, Artificial Sequence
  muFas tm-CD28
MLWIWAVLPLVLAGSQLRVHTQGTNSISESLKLRRRVRETDKNCSEGLYQGGPFCCQPCQPGKKKVEDCKMNGGTPTCAPCTEGKEYMDKNHYADKCRRCTLCDEEHGLEVETNCTLTQNTKCKCKPDFYCDSPGCEHCVRCASCEHGTLEPCTATSNTNCRKQSPRNRLWLLTILVLLIPLVFIYNSRRNRGGQSDYMNMTPRRPGLTRKPYQPYAPARDFAAYRP

SEQ ID NO: 119 - DNA, 711 bp, Artificial Sequence
  muFas-CD28tm
atgctgtggatctgggccgtgctgcctctggtgctggctggatcacagctgagagtgcacacccagggcaccaacagcatcagcgagagcctgaagctgagaagaagagtgcgcgagacagacaagaactgcagcgagggcctgtaccagggcggacccttctgctgtcagccttgccagcccggcaagaaaaaggtggaagattgcaagatgaacggcggcacccctacctgcgccccttgtacagagggcaaagagtacatggacaagaaccactacgccgacaagtgcagacggtgcaccctgtgcgacgaggaacacggcctggaagtggaaacaaactgcaccctgacccagaacaccaagtgcaagtgcaaacccgacttctactgcgacagccccggctgcgagcactgcgtcagatgtgcctcttgcgagcacggcaccctggaaccttgtaccgccaccagcaacaccaactgccggaagcagagccccagaaacagattctgggccctggtggtggtggccggcgtgctgttttgttacggcctgctcgtgaccgtggccctgtgcgtgatctggaccaacagcagaagaaacagaggcggccagagcgactacatgaacatgacccccagaaggcctggcctgaccagaaagccctaccagccttacgcccctgccagagacttcgccgcctacagacct

SEQ ID NO: 120 - protein, 237 aa, Artificial Sequence
  muFas-CD28tm
MLWIWAVLPLVLAGSQLRVHTQGTNSISESLKLRRRVRETDKNCSEGLYQGGPFCCQPCQPGKKKVEDCKMNGGTPTCAPCTEGKEYMDKNHYADKCRRCTLCDEEHGLEVETNCTLTQNTKCKCKPDFYCDSPGCEHCVRCASCEHGTLEPCTATSNTNCRKQSPRNRFWALVVVAGVLFCYGLLVTVALCVIWTNSRRNRGGQSDYMNMTPRRPGLTRKPYQPYAPARDFAAYRP

SEQ ID NO: 121 - DNA, 738 bp, Artificial Sequence
  muFas-CD28Cys
atgctgtggatctgggccgtgctgcctctggtgctggctggatcacagctgagagtgcacacccagggcaccaacagcatcagcgagagcctgaagctgagaagaagagtgcgcgagacagacaagaactgcagcgagggcctgtaccagggcggacccttctgctgtcagccttgccagcccggcaagaaaaaggtggaagattgcaagatgaacggcggcacccctacctgcgccccttgtacagagggcaaagagtacatggacaagaaccactacgccgacaagtgcagacggtgcaccctgtgcgacgaggaacacggcctggaagtggaaacaaactgcaccctgacccagaacaccaagtgcaagtgcaaacccgacttctactgcgacagccccggctgcgagcactgcgtcagatgtgcctcttgcgagcacggcaccctggaaccttgtaccgccaccagcaacaccaactgccggaagcagagccccagaaacagatgccacacccagagcagccccaagctgttctgggccctggtggtggtggccggcgtgctgttttgttacggcctgctcgtgaccgtggccctgtgcgtgatctggaccaacagcagaagaaacagaggcggccagagcgactacatgaacatgacccccagaaggcctggcctgaccagaaagccctaccagccttacgcccctgccagagacttcgccgcctacagacct

SEQ ID NO: 122 - protein, 246 aa, Artificial Sequence
  muFas-CD28Cys
MLWIWAVLPLVLAGSQLRVHTQGTNSISESLKLRRRVRETDKNCSEGLYQGGPFCCQPCQPGKKKVEDCKMNGGTPTCAPCTEGKEYMDKNHYADKCRRCTLCDEEHGLEVETNCTLTQNTKCKCKPDFYCDSPGCEHCVRCASCEHGTLEPCTATSNTNCRKQSPRNRCHTQSSPKLFWALVVVAGVLFCYGLLVTVALCVIWTNSRRNRGGQSDYMNMTPRRPGLTRKPYQPYAPARDFAAYRP

SEQ ID NO: 123 - DNA, 711 bp, Artificial Sequence
  muFas-9aas-CD28Cys
atgctgtggatctgggccgtgctgcctctggtgctggctggatcacagctgagagtgcacacccagggcaccaacagcatcagcgagagcctgaagctgagaagaagagtgcgcgagacagacaagaactgcagcgagggcctgtaccagggcggacccttctgctgtcagccttgccagcccggcaagaaaaaggtggaagattgcaagatgaacggcggcacccctacctgcgccccttgtacagagggcaaagagtacatggacaagaaccactacgccgacaagtgcagacggtgcaccctgtgcgacgaggaacacggcctggaagtggaaacaaactgcaccctgacccagaacaccaagtgcaagtgcaaacccgacttctactgcgacagccccggctgcgagcactgcgtcagatgtgcctcttgcgagcacggcaccctggaaccttgtaccgccaccagcaacaccaactgccacacccagagcagccccaagctgttctgggccctggtggtggtggccggcgtgctgttttgttacggcctgctcgtgaccgtggccctgtgcgtgatctggaccaacagcagaagaaacagaggcggccagagcgactacatgaacatgacccccagaaggcctggcctgaccagaaagccctaccagccttacgcccctgccagagacttcgccgcctacagacct

SEQ ID NO: 124 - protein, 237 aa, Artificial Sequence
  muFas-9aas-CD28Cys
MLWIWAVLPLVLAGSQLRVHTQGTNSISESLKLRRRVRETDKNCSEGLYQGGPFCCQPCQPGKKKVEDCKMNGGTPTCAPCTEGKEYMDKNHYADKCRRCTLCDEEHGLEVETNCTLTQNTKCKCKPDFYCDSPGCEHCVRCASCEHGTLEPCTATSNTNCHTQSSPKLFWALVVVAGVLFCYGLLVTVALCVIWTNSRRNRGGQSDYMNMTPRRPGLTRKPYQPYAPARDFAAYRP

SEQ ID NO: 125 - DNA, 693 bp, Artificial Sequence
  muPD1tm-CD28
atgtgggtgcgacaggtgccctggtctttcacctgggctgtgctgcagctgagctggcagtctggctggctgctggaagtgcctaacggcccttggagaagcctgaccttctaccccgcttggctgaccgtgtctgagggcgccaacgccaccttcacctgtagcctgagcaattggagcgaggacctgatgctgaactggaacagactgagccccagcaaccagaccgagaagcaggccgccttctgcaacggcctgtctcagcctgtgcaggacgccagattccagatcatccagctgcccaacagacacgacttccacatgaacatcctggacaccagaagaaacgacagcggcatctacctgtgcggcgccatcagcctgcaccccaaggccaagatcgaggaatctcctggcgccgagctggtcgtgaccgagagaatcctggaaacctccaccagataccccagccccagccctaagcccgagggcagatttcagggcatggtcatcggcatcatgagcgccctcgtgggcatcccagtgttgctgctgctggcctgggccctgaacagcagaagaaacagaggcggccagagcgactacatgaacatgacccccagaaggcctggcctgaccagaaagccctaccagccttacgcccctgccagagacttcgccgcctacagacct

SEQ ID NO: 126 - protein, 231 aa, Artificial Sequence
  muPD1tm-CD28
MWVRQVPWSFTWAVLQLSWQSGWLLEVPNGPWRSLTFYPAWLTVSEGANATFTCSLSNWSEDLMLNWNRLSPSNQTEKQAAFCNGLSQPVQDARFQIIQLPNRHDFHMNILDTRRNDSGIYLCGAISLHPKAKIEESPGAELVVTERILETSTRYPSPSPKPEGRFQGMVIGIMSALVGIPVLLLLAWALNSRRNRGGQSDYMNMTPRRPGLTRKPYQPYAPARDFAAYRP

SEQ ID NO: 127 - DNA, 711 bp, Artificial Sequence
  muPD1-CD28tm
atgtgggtgcgacaggtgccctggtctttcacctgggctgtgctgcagctgagctggcagtctggctggctgctggaagtgcctaacggcccttggagaagcctgaccttctaccccgcttggctgaccgtgtctgagggcgccaacgccaccttcacctgtagcctgagcaattggagcgaggacctgatgctgaactggaacagactgagccccagcaaccagaccgagaagcaggccgccttctgcaacggcctgtctcagcctgtgcaggacgccagattccagatcatccagctgcccaacagacacgacttccacatgaacatcctggacaccagaagaaacgacagcggcatctacctgtgcggcgccatcagcctgcaccccaaggccaagatcgaggaatctcctggcgccgagctggtcgtgaccgagagaatcctggaaacctccaccagataccccagccccagccctaagcccgagggcagatttcagggcatgttctgggccctggtggtggtggccggcgtgctgttttgttacggcctgctcgtgaccgtggccctgtgcgtgatctggaccaacagcagaagaaacagaggcggccagagcgactacatgaacatgacccccagaaggcctggcctgaccagaaagccctaccagccttacgcccctgccagagacttcgccgcctacagacct

SEQ ID NO: 128 - protein, 237 aa, Artificial Sequence
  muPD1-CD28tm
MWVRQVPWSFTWAVLQLSWQSGWLLEVPNGPWRSLTFYPAWLTVSEGANATFTCSLSNWSEDLMLNWNRLSPSNQTEKQAAFCNGLSQPVQDARFQIIQLPNRHDFHMNILDTRRNDSGIYLCGAISLHPKAKIEESPGAELVVTERILETSTRYPSPSPKPEGRFQGMFWALVVVAGVLFCYGLLVTVALCVIWTNSRRNRGGQSDYMNMTPRRPGLTRKPYQPYAPARDFAAYRP

SEQ ID NO: 129 - DNA, 738 bp, Artificial Sequence
  muPD1-CD28Cys
atgtgggtgcgacaggtgccctggtctttcacctgggctgtgctgcagctgagctggcagtctggctggctgctggaagtgcctaacggcccttggagaagcctgaccttctaccccgcttggctgaccgtgtctgagggcgccaacgccaccttcacctgtagcctgagcaattggagcgaggacctgatgctgaactggaacagactgagccccagcaaccagaccgagaagcaggccgccttctgcaacggcctgtctcagcctgtgcaggacgccagattccagatcatccagctgcccaacagacacgacttccacatgaacatcctggacaccagaagaaacgacagcggcatctacctgtgcggcgccatcagcctgcaccccaaggccaagatcgaggaatctcctggcgccgagctggtcgtgaccgagagaatcctggaaacctccaccagataccccagccccagccctaagcccgagggcagatttcagggcatgtgccacacccagagcagccccaagctgttctgggctctggtggtggtggccggcgtgctgttttgttacggcctgctcgtgaccgtggccctgtgcgtgatctggaccaacagcagacggaacagaggcggccagagcgactacatgaatatgacccccagaaggcctggcctgaccagaaagccctaccagccttacgcccctgccagagacttcgccgcctacagacct

SEQ ID NO: 130 - protein, 246 aa, Artificial Sequence
  muPD1-CD28Cys
MWVRQVPWSFTWAVLQLSWQSGWLLEVPNGPWRSLTFYPAWLTVSEGANATFTCSLSNWSEDLMLNWNRLSPSNQTEKQAAFCNGLSQPVQDARFQIIQLPNRHDFHMNILDTRRNDSGIYLCGAISLHPKAKIEESPGAELVVTERILETSTRYPSPSPKPEGRFQGMCHTQSSPKLFWALVVVAGVLFCYGLLVTVALCVIWTNSRRNRGGQSDYMNMTPRRPGLTRKPYQPYAPARDFAAYRP

SEQ ID NO: 131 - DNA, 711 bp, Artificial Sequence
  muPD1-9aas-CD28Cys
atgtgggtgcgacaggtgccctggtctttcacctgggctgtgctgcagctgagctggcagtctggctggctgctggaagtgcctaacggcccttggagaagcctgaccttctaccccgcttggctgaccgtgtctgagggcgccaacgccaccttcacctgtagcctgagcaattggagcgaggacctgatgctgaactggaacagactgagccccagcaaccagaccgagaagcaggccgccttctgcaacggcctgtctcagcctgtgcaggacgccagattccagatcatccagctgcccaacagacacgacttccacatgaacatcctggacaccagaagaaacgacagcggcatctacctgtgcggcgccatcagcctgcaccccaaggccaagatcgaggaatctcctggcgccgagctggtcgtgaccgagagaatcctggaaacctccaccagataccccagccccagcccttgccacacccagagcagccccaagctgttctgggctctggtggtggtggccggcgtgctgttttgttacggcctgctcgtgaccgtggccctgtgcgtgatctggaccaacagcagacggaacagaggcggccagagcgactacatgaatatgacccccagaaggcctggcctgaccagaaagccctaccagccttacgcccctgccagagacttcgccgcctacagacct

SEQ ID NO: 132 - protein, 237 aa, Artificial Sequence
  muPD1-9aas-CD28Cys
MWVRQVPWSFTWAVLQLSWQSGWLLEVPNGPWRSLTFYPAWLTVSEGANATFTCSLSNWSEDLMLNWNRLSPSNQTEKQAAFCNGLSQPVQDARFQIIQLPNRHDFHMNILDTRRNDSGIYLCGAISLHPKAKIEESPGAELVVTERILETSTRYPSPSPCHTQSSPKLFWALVVVAGVLFCYGLLVTVALCVIWTNSRRNRGGQSDYMNMTPRRPGLTRKPYQPYAPARDFAAYRP

SEQ ID NO: 133 - DNA, 675 bp, Artificial Sequence
  muPD1-21aas-CD28Cys
atgtgggtgcgacaggtgccctggtctttcacctgggctgtgctgcagctgagctggcagtctggctggctgctggaagtgcctaacggcccttggagaagcctgaccttctaccccgcttggctgaccgtgtctgagggcgccaacgccaccttcacctgtagcctgagcaattggagcgaggacctgatgctgaactggaacagactgagccccagcaaccagaccgagaagcaggccgccttctgcaacggcctgtctcagcctgtgcaggacgccagattccagatcatccagctgcccaacagacacgacttccacatgaacatcctggacaccagaagaaacgacagcggcatctacctgtgcggcgccatcagcctgcaccccaaggccaagatcgaggaatctcctggcgccgagctggtcgtgaccgagagaatctgccacacccagagcagccccaagctgttctgggctctggtggtggtggccggcgtgctgttttgttacggcctgctcgtgaccgtggccctgtgcgtgatctggaccaacagcagacggaacagaggcggccagagcgactacatgaatatgacccccagaaggcctggcctgaccagaaagccctaccagccttacgcccctgccagagacttcgccgcctacagacct

SEQ ID NO: 134 - protein, 225 aa, Artificial Sequence
  muPD1-21aas-CD28Cys
MWVRQVPWSFTWAVLQLSWQSGWLLEVPNGPWRSLTFYPAWLTVSEGANATFTCSLSNWSEDLMLNWNRLSPSNQTEKQAAFCNGLSQPVQDARFQIIQLPNRHDFHMNILDTRRNDSGIYLCGAISLHPKAKIEESPGAELVVTERICHTQSSPKLFWALVVVAGVLFCYGLLVTVALCVIWTNSRRNRGGQSDYMNMTPRRPGLTRKPYQPYAPARDFAAYRP

SEQ ID NO: 135 - DNA, 1512 bp, Artificial Sequence
  muLag3tm-CD28
atgagagaggacctgctgctgggctttctgctgctgggactgctgtgggaggcccctgtggtgtcatctggccctggcaaagaactgcccgtcgtgtgggctcaggaaggcgctcctgtgcatctgccctgcagcctgaagtcccccaacctggaccccaacttcctgagaagaggcggcgtgatctggcagcaccagcctgattctggccagcccacacctatccctgccctggatctgcaccagggcatgcctagccctagacagcctgcccctggcagatacaccgtgctgtctgtggctcctggcggcctgagaagtggcagacagcctctgcaccctcacgtgcagctggaagagaggggactgcagaggggcgacttcagcctgtggctgaggcctgccctgagaacagatgccggcgagtaccacgctaccgtgcggctgcctaacagagccctgagctgctccctgagactgagagtgggccaggccagcatgatcgcctctccatctggcgtgctgaagctgagcgactgggtgctgctgaactgcagcttctccagacccgacagacccgtgtccgtgcactggttccagggacagaacagagtgcccgtgtacaacagccccagacacttcctggccgagacattcctgctgctgccccaggtgtcccctctggactctggcacatggggctgcgtgctgacatacagggacggcttcaacgtgtccatcacctacaacctgaaggtgctgggcctggaacccgtggctcctctgacagtgtacgccgccgagggcagcagagtggaactgccttgtcatctgccacccggcgtgggcacaccttctctgctgatcgccaagtggacccctccaggcggaggacctgaactgccagtggctggcaagagcggcaacttcaccctgcacctggaagcagtgggcctggctcaggccggcacctacacctgtagcatccatctgcagggccagcagctgaacgccaccgtgacactggccgtgatcaccgtgacccccaagagctttggcctgcctggctccagaggcaagctgctgtgtgaagtgacccccgccagcggcaaagaaagattcgtgtggcggcctctgaacaacctgagcagatcctgcccaggccccgtgctggaaatccaggaagccagactgctggccgagcggtggcagtgccagctgtatgagggacagcgactgctgggcgccactgtgtacgctgctgagtctagctctggcgcccacagcgccagaagaatcagcggcgatctgaagggcggccacctggtgctggtgctgatcctgggcgctctgagcctgttcctgctggtggctggcgctttcggctttaacagcagaagaaacagaggcggccagagcgactacatgaacatgacccccagaaggcctggcctgaccagaaagccctaccagccttacgcccctgccagagacttcgccgcctacagacct

SEQ ID NO: 136 - protein, 504 aa, Artificial Sequence
  muLag3tm-CD28
MREDLLLGFLLLGLLWEAPVVSSGPGKELPVVWAQEGAPVHLPCSLKSPNLDPNFLRRGGVIWQHQPDSGQPTPIPALDLHQGMPSPRQPAPGRYTVLSVAPGGLRSGRQPLHPHVQLEERGLQRGDFSLWLRPALRTDAGEYHATVRLPNRALSCSLRLRVGQASMIASPSGVLKLSDWVLLNCSFSRPDRPVSVHWFQGQNRVPVYNSPRHFLAETFLLLPQVSPLDSGTWGCVLTYRDGFNVSITYNLKVLGLEPVAPLTVYAAEGSRVELPCHLPPGVGTPSLLIAKWTPPGGGPELPVAGKSGNFTLHLEAVGLAQAGTYTCSIHLQGQQLNATVTLAVITVTPKSFGLPGSRGKLLCEVTPASGKERFVWRPLNNLSRSCPGPVLEIQEARLLAERWQCQLYEGQRLLGATVYAAESSSGAHSARRISGDLKGGHLVLVLILGALSLFLLVAGAFGFNSRRNRGGQSDYMNMTPRRPGLTRKPYQPYAPARDFAAYRP

SEQ ID NO: 137 - DNA, 1530 bp, Artificial Sequence
  muLag3-CD28tm
atgagagaggacctgctgctgggctttctgctgctgggactgctgtgggaggcccctgtggtgtcatctggccctggcaaagaactgcccgtcgtgtgggctcaggaaggcgctcctgtgcatctgccctgcagcctgaagtcccccaacctggaccccaacttcctgagaagaggcggcgtgatctggcagcaccagcctgattctggccagcccacacctatccctgccctggatctgcaccagggcatgcctagccctagacagcctgcccctggcagatacaccgtgctgtctgtggctcctggcggcctgagaagtggcagacagcctctgcaccctcacgtgcagctggaagagaggggactgcagaggggcgacttcagcctgtggctgaggcctgccctgagaacagatgccggcgagtaccacgctaccgtgcggctgcctaacagagccctgagctgctccctgagactgagagtgggccaggccagcatgatcgcctctccatctggcgtgctgaagctgagcgactgggtgctgctgaactgcagcttctccagacccgacagacccgtgtccgtgcactggttccagggacagaacagagtgcccgtgtacaacagccccagacacttcctggccgagacattcctgctgctgccccaggtgtcccctctggactctggcacatggggctgcgtgctgacatacagggacggcttcaacgtgtccatcacctacaacctgaaggtgctgggcctggaacccgtggctcctctgacagtgtacgccgccgagggcagcagagtggaactgccttgtcatctgccacccggcgtgggcacaccttctctgctgatcgccaagtggacccctccaggcggaggacctgaactgccagtggctggcaagagcggcaacttcaccctgcacctggaagcagtgggcctggctcaggccggcacctacacctgtagcatccatctgcagggccagcagctgaacgccaccgtgacactggccgtgatcaccgtgacccccaagagctttggcctgcctggctccagaggcaagctgctgtgtgaagtgacccccgccagcggcaaagaaagattcgtgtggcggcctctgaacaacctgagcagatcctgcccaggccccgtgctggaaatccaggaagccagactgctggccgagcggtggcagtgccagctgtatgagggacagcgactgctgggcgccactgtgtacgctgctgagtctagctctggcgcccacagcgccagaagaatcagcggcgatctgaagggcggccacctgttctgggccctggtggtggtggccggcgtgctgttttgttacggcctgctcgtgaccgtggccctgtgcgtgatctggaccaacagcagaagaaacagaggcggccagagcgactacatgaacatgacccccagaaggcctggcctgaccagaaagccctaccagccttacgcccctgccagagacttcgccgcctacagacct

SEQ ID NO: 138 - protein, 510 aa, Artificial Sequence
  muLag3-CD28tm
MREDLLLGFLLLGLLWEAPVVSSGPGKELPVVWAQEGAPVHLPCSLKSPNLDPNFLRRGGVIWQHQPDSGQPTPIPALDLHQGMPSPRQPAPGRYTVLSVAPGGLRSGRQPLHPHVQLEERGLQRGDFSLWLRPALRTDAGEYHATVRLPNRALSCSLRLRVGQASMIASPSGVLKLSDWVLLNCSFSRPDRPVSVHWFQGQNRVPVYNSPRHFLAETFLLLPQVSPLDSGTWGCVLTYRDGFNVSITYNLKVLGLEPVAPLTVYAAEGSRVELPCHLPPGVGTPSLLIAKWTPPGGGPELPVAGKSGNFTLHLEAVGLAQAGTYTCSIHLQGQQLNATVTLAVITVTPKSFGLPGSRGKLLCEVTPASGKERFVWRPLNNLSRSCPGPVLEIQEARLLAERWQCQLYEGQRLLGATVYAAESSSGAHSARRISGDLKGGHLFWALVVVAGVLFCYGLLVTVALCVIWTNSRRNRGGQSDYMNMTPRRPGLTRKPYQPYAPARDFAAYRP

SEQ ID NO: 139 - DNA, 1557 bp, Artificial Sequence
  muLag3-CD28Cys
atgagagaggacctgctgctgggctttctgctgctgggactgctgtgggaggcccctgtggtgtcatctggccctggcaaagaactgcccgtcgtgtgggctcaggaaggcgctcctgtgcatctgccctgcagcctgaagtcccccaacctggaccccaacttcctgagaagaggcggcgtgatctggcagcaccagcctgattctggccagcccacacctatccctgccctggatctgcaccagggcatgcctagccctagacagcctgcccctggcagatacaccgtgctgtctgtggctcctggcggcctgagaagtggcagacagcctctgcaccctcacgtgcagctggaagagaggggactgcagaggggcgacttcagcctgtggctgaggcctgccctgagaacagatgccggcgagtaccacgctaccgtgcggctgcctaacagagccctgagctgctccctgagactgagagtgggccaggccagcatgatcgcctctccatctggcgtgctgaagctgagcgactgggtgctgctgaactgcagcttctccagacccgacagacccgtgtccgtgcactggttccagggacagaacagagtgcccgtgtacaacagccccagacacttcctggccgagacattcctgctgctgccccaggtgtcccctctggactctggcacatggggctgcgtgctgacatacagggacggcttcaacgtgtccatcacctacaacctgaaggtgctgggcctggaacccgtggctcctctgacagtgtacgccgccgagggcagcagagtggaactgccttgtcatctgccacccggcgtgggcacaccttctctgctgatcgccaagtggacccctccaggcggaggacctgaactgccagtggctggcaagagcggcaacttcaccctgcacctggaagcagtgggcctggctcaggccggcacctacacctgtagcatccatctgcagggccagcagctgaacgccaccgtgacactggccgtgatcaccgtgacccccaagagctttggcctgcctggctccagaggcaagctgctgtgtgaagtgacccccgccagcggcaaagaaagattcgtgtggcggcctctgaacaacctgagcagatcctgcccaggccccgtgctggaaatccaggaagccagactgctggccgagcggtggcagtgccagctgtatgagggacagcgactgctgggcgccactgtgtacgctgctgagtctagctctggcgcccacagcgccagaagaatcagcggcgatctgaagggcggccacctgtgccacacccagagcagccccaagctgttctgggccctggtggtggtggccggcgtgctgttttgttacggcctgctcgtgaccgtggccctgtgcgtgatctggaccaacagcagaagaaacagaggcggccagagcgactacatgaacatgacccccagaaggcctggcctgaccagaaagccctaccagccttacgcccctgccagagacttcgccgcctacagacct

SEQ ID NO: 140 - protein, 519 aa, Artificial Sequence
  muLag3-CD28Cys
MREDLLLGFLLLGLLWEAPVVSSGPGKELPVVWAQEGAPVHLPCSLKSPNLDPNFLRRGGVIWQHQPDSGQPTPIPALDLHQGMPSPRQPAPGRYTVLSVAPGGLRSGRQPLHPHVQLEERGLQRGDFSLWLRPALRTDAGEYHATVRLPNRALSCSLRLRVGQASMIASPSGVLKLSDWVLLNCSFSRPDRPVSVHWFQGQNRVPVYNSPRHFLAETFLLLPQVSPLDSGTWGCVLTYRDGFNVSITYNLKVLGLEPVAPLTVYAAEGSRVELPCHLPPGVGTPSLLIAKWTPPGGGPELPVAGKSGNFTLHLEAVGLAQAGTYTCSIHLQGQQLNATVTLAVITVTPKSFGLPGSRGKLLCEVTPASGKERFVWRPLNNLSRSCPGPVLEIQEARLLAERWQCQLYEGQRLLGATVYAAESSSGAHSARRISGDLKGGHLCHTQSSPKLFWALVVVAGVLFCYGLLVTVALCVIWTNSRRNRGGQSDYMNMTPRRPGLTRKPYQPYAPARDFAAYRP

SEQ ID NO: 141 - DNA, 1530 bp, Artificial Sequence
  muLag3-9aas-CD28Cys
atgagagaggacctgctgctgggctttctgctgctgggactgctgtgggaggcccctgtggtgtcatctggccctggcaaagaactgcccgtcgtgtgggctcaggaaggcgctcctgtgcatctgccctgcagcctgaagtcccccaacctggaccccaacttcctgagaagaggcggcgtgatctggcagcaccagcctgattctggccagcccacacctatccctgccctggatctgcaccagggcatgcctagccctagacagcctgcccctggcagatacaccgtgctgtctgtggctcctggcggcctgagaagtggcagacagcctctgcaccctcacgtgcagctggaagagaggggactgcagaggggcgacttcagcctgtggctgaggcctgccctgagaacagatgccggcgagtaccacgctaccgtgcggctgcctaacagagccctgagctgctccctgagactgagagtgggccaggccagcatgatcgcctctccatctggcgtgctgaagctgagcgactgggtgctgctgaactgcagcttctccagacccgacagacccgtgtccgtgcactggttccagggacagaacagagtgcccgtgtacaacagccccagacacttcctggccgagacattcctgctgctgccccaggtgtcccctctggactctggcacatggggctgcgtgctgacatacagggacggcttcaacgtgtccatcacctacaacctgaaggtgctgggcctggaacccgtggctcctctgacagtgtacgccgccgagggcagcagagtggaactgccttgtcatctgccacccggcgtgggcacaccttctctgctgatcgccaagtggacccctccaggcggaggacctgaactgccagtggctggcaagagcggcaacttcaccctgcacctggaagcagtgggcctggctcaggccggcacctacacctgtagcatccatctgcagggccagcagctgaacgccaccgtgacactggccgtgatcaccgtgacccccaagagctttggcctgcctggctccagaggcaagctgctgtgtgaagtgacccccgccagcggcaaagaaagattcgtgtggcggcctctgaacaacctgagcagatcctgcccaggccccgtgctggaaatccaggaagccagactgctggccgagcggtggcagtgccagctgtatgagggacagcgactgctgggcgccactgtgtacgctgctgagtctagctctggcgcccacagcgccagaagaatctgccacacccagagcagccccaagctgttctgggccctggtggtggtggccggcgtgctgttttgttacggcctgctcgtgaccgtggccctgtgcgtgatctggaccaacagcagaagaaacagaggcggccagagcgactacatgaacatgacccccagaaggcctggcctgaccagaaagccctaccagccttacgcccctgccagagacttcgccgcctacagacct

SEQ ID NO: 142 - protein, 510 aa, Artificial Sequence
  muLag3-9aas-CD28Cys
MREDLLLGFLLLGLLWEAPVVSSGPGKELPVVWAQEGAPVHLPCSLKSPNLDPNFLRRGGVIWQHQPDSGQPTPIPALDLHQGMPSPRQPAPGRYTVLSVAPGGLRSGRQPLHPHVQLEERGLQRGDFSLWLRPALRTDAGEYHATVRLPNRALSCSLRLRVGQASMIASPSGVLKLSDWVLLNCSFSRPDRPVSVHWFQGQNRVPVYNSPRHFLAETFLLLPQVSPLDSGTWGCVLTYRDGFNVSITYNLKVLGLEPVAPLTVYAAEGSRVELPCHLPPGVGTPSLLIAKWTPPGGGPELPVAGKSGNFTLHLEAVGLAQAGTYTCSIHLQGQQLNATVTLAVITVTPKSFGLPGSRGKLLCEVTPASGKERFVWRPLNNLSRSCPGPVLEIQEARLLAERWQCQLYEGQRLLGATVYAAESSSGAHSARRICHTQSSPKLFWALVVVAGVLFCYGLLVTVALCVIWTNSRRNRGGQSDYMNMTPRRPGLTRKPYQPYAPARDFAAYRP

SEQ ID NO: 143 - DNA, 765 bp, Artificial Sequence
  muTim3tm-CD28
atgttcagcggcctgaccctgaactgcgtgctcctgctgctgcagctgctgctggccagaagcctggaaaacgcctacgtgttcgaagtgggcaagaacgcctacctgccctgcagctacaccctgtctacacctggcgccctggtgcctatgtgttggggcaagggcttctgcccttggagccagtgcaccaacgagctgctgagaaccgacgagagaaacgtgacctaccagaagtccagcagataccagctgaagggcgacctgaacaagggcgacgtgtccctgatcatcaagaacgtgaccctggacgaccacggcacctactgctgcagaatccagttccccggcctgatgaacgacaagaagctggaactgaagctggacatcaaggccgccaaagtgacccctgcccagacagcccacggcgactctacaacagccagccccagaaccctgaccaccgagaggaacggcagcgagacacagaccctcgtgacactgcacaacaacaacggcaccaagatcagcacctgggccgacgagatcaaggacagcggcgagacaatcagaaccgccatccacatcggcgtgggcgtgtccgctggactgacactggctctgatcatcggagtgctgatcaacagcagaagaaacagaggcggccagagcgactacatgaacatgacccccagaaggcctggcctgaccagaaagccctaccagccttacgcccctgccagagacttcgccgcctacagacct

SEQ ID NO: 144 - protein, 255 aa, Artificial Sequence
  muTim3tm-CD28
MFSGLTLNCVLLLLQLLLARSLENAYVFEVGKNAYLPCSYTLSTPGALVPMCWGKGFCPWSQCTNELLRTDERNVTYQKSSRYQLKGDLNKGDVSLIIKNVTLDDHGTYCCRIQFPGLMNDKKLELKLDIKAAKVTPAQTAHGDSTTASPRTLTTERNGSETQTLVTLHNNNGTKISTWADEIKDSGETIRTAIHIGVGVSAGLTLALIIGVLINSRRNRGGQSDYMNMTPRRPGLTRKPYQPYAPARDFAAYRP

SEQ ID NO: 145 - DNA, 783 bp, Artificial Sequence
  muTim3-CD28tm
atgttcagcggcctgaccctgaactgcgtgctcctgctgctgcagctgctgctggccagaagcctggaaaacgcctacgtgttcgaagtgggcaagaacgcctacctgccctgcagctacaccctgtctacacctggcgccctggtgcctatgtgttggggcaagggcttctgcccttggagccagtgcaccaacgagctgctgagaaccgacgagagaaacgtgacctaccagaagtccagcagataccagctgaagggcgacctgaacaagggcgacgtgtccctgatcatcaagaacgtgaccctggacgaccacggcacctactgctgcagaatccagttccccggcctgatgaacgacaagaagctggaactgaagctggacatcaaggccgccaaagtgacccctgcccagacagcccacggcgactctacaacagccagccccagaaccctgaccaccgagaggaacggcagcgagacacagaccctcgtgacactgcacaacaacaacggcaccaagatcagcacctgggccgacgagatcaaggacagcggcgagacaatcagaaccgccttctgggccctggtggtggtggccggcgtgctgttttgttacggcctgctcgtgaccgtggccctgtgcgtgatctggaccaacagcagaagaaacagaggcggccagagcgactacatgaacatgacccccagaaggcctggcctgaccagaaagccctaccagccttacgcccctgccagagacttcgccgcctacagacct

SEQ ID NO: 146 - protein, 261 aa, Artificial Sequence
  muTim3-CD28tm
MFSGLTLNCVLLLLQLLLARSLENAYVFEVGKNAYLPCSYTLSTPGALVPMCWGKGFCPWSQCTNELLRTDERNVTYQKSSRYQLKGDLNKGDVSLIIKNVTLDDHGTYCCRIQFPGLMNDKKLELKLDIKAAKVTPAQTAHGDSTTASPRTLTTERNGSETQTLVTLHNNNGTKISTWADEIKDSGETIRTAFWALVVVAGVLFCYGLLVTVALCVIWTNSRRNRGGQSDYMNMTPRRPGLTRKPYQPYAPARDFAAYRP

SEQ ID NO: 147 - DNA, 810 bp, Artificial Sequence
  muTim3-CD28Cys
atgttcagcggcctgaccctgaactgcgtgctcctgctgctgcagctgctgctggccagaagcctggaaaacgcctacgtgttcgaagtgggcaagaacgcctacctgccctgcagctacaccctgtctacacctggcgccctggtgcctatgtgttggggcaagggcttctgcccttggagccagtgcaccaacgagctgctgagaaccgacgagagaaacgtgacctaccagaagtccagcagataccagctgaagggcgacctgaacaagggcgacgtgtccctgatcatcaagaacgtgaccctggacgaccacggcacctactgctgcagaatccagttccccggcctgatgaacgacaagaagctggaactgaagctggacatcaaggccgccaaagtgacccctgcccagacagcccacggcgactctacaacagccagccccagaaccctgaccaccgagaggaacggcagcgagacacagaccctcgtgacactgcacaacaacaacggcaccaagatcagcacctgggccgacgagatcaaggacagcggcgagacaatcagaaccgcctgccacacccagagcagccccaagctgttctgggccctggtggtggtggccggcgtgctgttttgttacggcctgctcgtgaccgtggccctgtgcgtgatctggaccaacagcagaagaaacagaggcggccagagcgactacatgaacatgacccccagaaggcctggcctgaccagaaagccctaccagccttacgcccctgccagagacttcgccgcctacagacct

SEQ ID NO: 148 - protein, 270 aa, Artificial Sequence
  muTim3-CD28Cys
MFSGLTLNCVLLLLQLLLARSLENAYVFEVGKNAYLPCSYTLSTPGALVPMCWGKGFCPWSQCTNELLRTDERNVTYQKSSRYQLKGDLNKGDVSLIIKNVTLDDHGTYCCRIQFPGLMNDKKLELKLDIKAAKVTPAQTAHGDSTTASPRTLTTERNGSETQTLVTLHNNNGTKISTWADEIKDSGETIRTACHTQSSPKLFWALVVVAGVLFCYGLLVTVALCVIWTNSRRNRGGQSDYMNMTPRRPGLTRKPYQPYAPARDFAAYRP

SEQ ID NO: 149 - DNA, 783 bp, Artificial Sequence
  muTim3-9aas-CD28Cys
atgttcagcggcctgaccctgaactgcgtgctcctgctgctgcagctgctgctggccagaagcctggaaaacgcctacgtgttcgaagtgggcaagaacgcctacctgccctgcagctacaccctgtctacacctggcgccctggtgcctatgtgttggggcaagggcttctgcccttggagccagtgcaccaacgagctgctgagaaccgacgagagaaacgtgacctaccagaagtccagcagataccagctgaagggcgacctgaacaagggcgacgtgtccctgatcatcaagaacgtgaccctggacgaccacggcacctactgctgcagaatccagttccccggcctgatgaacgacaagaagctggaactgaagctggacatcaaggccgccaaagtgacccctgcccagacagcccacggcgactctacaacagccagccccagaaccctgaccaccgagaggaacggcagcgagacacagaccctcgtgacactgcacaacaacaacggcaccaagatcagcacctgggccgacgagatcaagtgccacacccagagcagccccaagctgttctgggccctggtggtggtggccggcgtgctgttttgttacggcctgctcgtgaccgtggccctgtgcgtgatctggaccaacagcagaagaaacagaggcggccagagcgactacatgaacatgacccccagaaggcctggcctgaccagaaagccctaccagccttacgcccctgccagagacttcgccgcctacagacct

SEQ ID NO: 150 - protein, 261 aa, Artificial Sequence
  muTim3-9aas-CD28Cys
MFSGLTLNCVLLLLQLLLARSLENAYVFEVGKNAYLPCSYTLSTPGALVPMCWGKGFCPWSQCTNELLRTDERNVTYQKSSRYQLKGDLNKGDVSLIIKNVTLDDHGTYCCRIQFPGLMNDKKLELKLDIKAAKVTPAQTAHGDSTTASPRTLTTERNGSETQTLVTLHNNNGTKISTWADEIKCHTQSSPKLFWALVVVAGVLFCYGLLVTVALCVIWTNSRRNRGGQSDYMNMTPRRPGLTRKPYQPYAPARDFAAYRP

SEQ ID NO: 151 - DNA, 1536 bp, Artificial Sequence
  huLag3tm-CD28
atgtgggaagcgcagtttcttggacttctttttctccagccgctgtgggttgcgccagtaaagccgctccaacccggtgcagaggttccggtagtgtgggcgcaagagggtgcaccagcgcagctcccctgcagtccgacgattccgctgcaagatttgtcactgcttagaagggcgggcgtaacgtggcagcaccaaccggatagtggccctccggctgcagcaccagggcacccactcgcccccggccctcatcccgcagcaccgagcagctggggtcctagaccacgcagatatacagtactctcagtaggtcccggcggcctgcggtccggtcgcttgccccttcaacctagagtacagctggatgaaagaggtcgacaacggggtgatttctccctctggttgaggcctgcacgacgagcagatgctggggagtatagggctgccgtacacctgcgagaccgcgcacttagttgtagactccggctccggctgggacaggcctctatgacagcgtccccccctgggtccctgcgagcctctgattgggtaatactcaactgctcattttctcggccagatcgccccgctagtgttcattggttccgaaatcgcggccaaggtcgcgtgcctgttcgagaatctccacaccaccatttggcggagtcttttctttttctgcctcaggtctcccctatggactctggaccgtggggctgtattttgacatatcgggatgggtttaacgtgagtataatgtataatctcactgtcttgggtcttgagccacctacgccgctgacggtgtacgcgggagccggcagccgggttggtctgccctgcaggctgcctgcaggagtcgggacaaggtcattccttacagcaaagtggaccccgccaggtggggggcccgacctccttgtaacgggagataatggagatttcactctgagacttgaggatgtctctcaagctcaggctgggacttatacatgtcacattcacttgcaagaacagcagttgaatgcgacggttaccctggctatcataacagtaacacctaaatctttcggtagtccgggtagcctgggcaaactgttgtgtgaggtaacccccgtgtcaggtcaagagcggttcgtctggagctcattggacactccctcacagcgatcctttagcggaccctggctcgaagcccaagaagcccagctgctttcccaaccatggcagtgtcaactctatcagggtgagcgccttctcggtgcggctgtctacttcaccgaattgtcctctccgggagcgcaaagaagtggacgcgccccaggggccctcccggcaggacaccttctgctgtttttgattttgggggtacttagtttgctgctgcttgtcacaggcgctttcggtttccgcagcaagcggagcagaggcggccacagcgactacatgaacatgacccctagacggcctggccccaccagaaagcactaccagccctacgcccctccccgggactttgccgcctacagaagc

SEQ ID NO: 152 - protein, 512 aa, Artificial Sequence
  huLag3tm-CD28
MWEAQFLGLLFLQPLWVAPVKPLQPGAEVPVVWAQEGAPAQLPCSPTIPLQDLSLLRRAGVTWQHQPDSGPPAAAPGHPLAPGPHPAAPSSWGPRPRRYTVLSVGPGGLRSGRLPLQPRVQLDERGRQRGDFSLWLRPARRADAGEYRAAVHLRDRALSCRLRLRLGQASMTASPPGSLRASDWVILNCSFSRPDRPASVHWFRNRGQGRVPVRESPHHHLAESFLFLPQVSPMDSGPWGCILTYRDGFNVSIMYNLTVLGLEPPTPLTVYAGAGSRVGLPCRLPAGVGTRSFLTAKWTPPGGGPDLLVTGDNGDFTLRLEDVSQAQAGTYTCHIHLQEQQLNATVTLAIITVTPKSFGSPGSLGKLLCEVTPVSGQERFVWSSLDTPSQRSFSGPWLEAQEAQLLSQPWQCQLYQGERLLGAAVYFTELSSPGAQRSGRAPGALPAGHLLLFLILGVLSLLLLVTGAFGFRSKRSRGGHSDYMNMTPRRPGPTRKHYQPYAPPRDFAAYRS

SEQ ID NO: 153 - DNA, 1350 bp, Artificial Sequence
  huLag3 ectodomain
atgtgggaagcgcagtttcttggacttctttttctccagccgctgtgggttgcgccagtaaagccgctccaacccggtgcagaggttccggtagtgtgggcgcaagagggtgcaccagcgcagctcccctgcagtccgacgattccgctgcaagatttgtcactgcttagaagggcgggcgtaacgtggcagcaccaaccggatagtggccctccggctgcagcaccagggcacccactcgcccccggccctcatcccgcagcaccgagcagctggggtcctagaccacgcagatatacagtactctcagtaggtcccggcggcctgcggtccggtcgcttgccccttcaacctagagtacagctggatgaaagaggtcgacaacggggtgatttctccctctggttgaggcctgcacgacgagcagatgctggggagtatagggctgccgtacacctgcgagaccgcgcacttagttgtagactccggctccggctgggacaggcctctatgacagcgtccccccctgggtccctgcgagcctctgattgggtaatactcaactgctcattttctcggccagatcgccccgctagtgttcattggttccgaaatcgcggccaaggtcgcgtgcctgttcgagaatctccacaccaccatttggcggagtcttttctttttctgcctcaggtctcccctatggactctggaccgtggggctgtattttgacatatcgggatgggtttaacgtgagtataatgtataatctcactgtcttgggtcttgagccacctacgccgctgacggtgtacgcgggagccggcagccgggttggtctgccctgcaggctgcctgcaggagtcgggacaaggtcattccttacagcaaagtggaccccgccaggtggggggcccgacctccttgtaacgggagataatggagatttcactctgagacttgaggatgtctctcaagctcaggctgggacttatacatgtcacattcacttgcaagaacagcagttgaatgcgacggttaccctggctatcataacagtaacacctaaatctttcggtagtccgggtagcctgggcaaactgttgtgtgaggtaacccccgtgtcaggtcaagagcggttcgtctggagctcattggacactccctcacagcgatcctttagcggaccctggctcgaagcccaagaagcccagctgctttcccaaccatggcagtgtcaactctatcagggtgagcgccttctcggtgcggctgtctacttcaccgaattgtcctctccgggagcgcaaagaagtggacgcgccccaggggccctcccggcaggacacctt

SEQ ID NO: 154 - protein, 450 aa, Artificial Sequence
  huLag3 ectodomain
MWEAQFLGLLFLQPLWVAPVKPLQPGAEVPVVWAQEGAPAQLPCSPTIPLQDLSLLRRAGVTWQHQPDSGPPAAAPGHPLAPGPHPAAPSSWGPRPRRYTVLSVGPGGLRSGRLPLQPRVQLDERGRQRGDFSLWLRPARRADAGEYRAAVHLRDRALSCRLRLRLGQASMTASPPGSLRASDWVILNCSFSRPDRPASVHWFRNRGQGRVPVRESPHHHLAESFLFLPQVSPMDSGPWGCILTYRDGFNVSIMYNLTVLGLEPPTPLTVYAGAGSRVGLPCRLPAGVGTRSFLTAKWTPPGGGPDLLVTGDNGDFTLRLEDVSQAQAGTYTCHIHLQEQQLNATVTLAIITVTPKSFGSPGSLGKLLCEVTPVSGQERFVWSSLDTPSQRSFSGPWLEAQEAQLLSQPWQCQLYQGERLLGAAVYFTELSSPGAQRSGRAPGALPAGHL

SEQ ID NO: 155 - DNA, 63 bp, Artificial Sequence
  huLag3 transmembrane domain
ctgctgtttttgattttgggggtacttagtttgctgctgcttgtcacaggcgctttcggtttc

SEQ ID NO: 156 - protein, 21 aa, Artificial Sequence
  huLag3 transmembrane domain
LLFLILGVLSLLLLVTGAFGF

SEQ ID NO: 157 - DNA, 1554 bp, Artificial Sequence
  huLag3-CD28tm
atgtgggaagcgcagtttcttggacttctttttctccagccgctgtgggttgcgccagtaaagccgctccaacccggtgcagaggttccggtagtgtgggcgcaagagggtgcaccagcgcagctcccctgcagtccgacgattccgctgcaagatttgtcactgcttagaagggcgggcgtaacgtggcagcaccaaccggatagtggccctccggctgcagcaccagggcacccactcgcccccggccctcatcccgcagcaccgagcagctggggtcctagaccacgcagatatacagtactctcagtaggtcccggcggcctgcggtccggtcgcttgccccttcaacctagagtacagctggatgaaagaggtcgacaacggggtgatttctccctctggttgaggcctgcacgacgagcagatgctggggagtatagggctgccgtacacctgcgagaccgcgcacttagttgtagactccggctccggctgggacaggcctctatgacagcgtccccccctgggtccctgcgagcctctgattgggtaatactcaactgctcattttctcggccagatcgccccgctagtgttcattggttccgaaatcgcggccaaggtcgcgtgcctgttcgagaatctccacaccaccatttggcggagtcttttctttttctgcctcaggtctcccctatggactctggaccgtggggctgtattttgacatatcgggatgggtttaacgtgagtataatgtataatctcactgtcttgggtcttgagccacctacgccgctgacggtgtacgcgggagccggcagccgggttggtctgccctgcaggctgcctgcaggagtcgggacaaggtcattccttacagcaaagtggaccccgccaggtggggggcccgacctccttgtaacgggagataatggagatttcactctgagacttgaggatgtctctcaagctcaggctgggacttatacatgtcacattcacttgcaagaacagcagttgaatgcgacggttaccctggctatcataacagtaacacctaaatctttcggtagtccgggtagcctgggcaaactgttgtgtgaggtaacccccgtgtcaggtcaagagcggttcgtctggagctcattggacactccctcacagcgatcctttagcggaccctggctcgaagcccaagaagcccagctgctttcccaaccatggcagtgtcaactctatcagggtgagcgccttctcggtgcggctgtctacttcaccgaattgtcctctccgggagcgcaaagaagtggacgcgccccaggggccctcccggcaggacaccttttctgggtgctggtggtggtcggaggcgtgctggcctgctacagcctgctggtcaccgtggccttcatcatcttttgggtccgcagcaagcggagcagaggcggccacagcgactacatgaacatgacccctagacggcctggccccaccagaaagcactaccagccctacgcccctccccgggactttgccgcctacagaagc

SEQ ID NO: 158 - protein, 518 aa, Artificial Sequence
  huLag3-CD28tm
MWEAQFLGLLFLQPLWVAPVKPLQPGAEVPVVWAQEGAPAQLPCSPTIPLQDLSLLRRAGVTWQHQPDSGPPAAAPGHPLAPGPHPAAPSSWGPRPRRYTVLSVGPGGLRSGRLPLQPRVQLDERGRQRGDFSLWLRPARRADAGEYRAAVHLRDRALSCRLRLRLGQASMTASPPGSLRASDWVILNCSFSRPDRPASVHWFRNRGQGRVPVRESPHHHLAESFLFLPQVSPMDSGPWGCILTYRDGFNVSIMYNLTVLGLEPPTPLTVYAGAGSRVGLPCRLPAGVGTRSFLTAKWTPPGGGPDLLVTGDNGDFTLRLEDVSQAQAGTYTCHIHLQEQQLNATVTLAIITVTPKSFGSPGSLGKLLCEVTPVSGQERFVWSSLDTPSQRSFSGPWLEAQEAQLLSQPWQCQLYQGERLLGAAVYFTELSSPGAQRSGRAPGALPAGHLFWVLVVVGGVLACYSLLVTVAFIIFWVRSKRSRGGHSDYMNMTPRRPGPTRKHYQPYAPPRDFAAYRS

SEQ ID NO: 159 - DNA, 1554 bp, Artificial Sequence
  huLag3-12aas-CD28Cys
atgtgggaagcgcagtttcttggacttctttttctccagccgctgtgggttgcgccagtaaagccgctccaacccggtgcagaggttccggtagtgtgggcgcaagagggtgcaccagcgcagctcccctgcagtccgacgattccgctgcaagatttgtcactgcttagaagggcgggcgtaacgtggcagcaccaaccggatagtggccctccggctgcagcaccagggcacccactcgcccccggccctcatcccgcagcaccgagcagctggggtcctagaccacgcagatatacagtactctcagtaggtcccggcggcctgcggtccggtcgcttgccccttcaacctagagtacagctggatgaaagaggtcgacaacggggtgatttctccctctggttgaggcctgcacgacgagcagatgctggggagtatagggctgccgtacacctgcgagaccgcgcacttagttgtagactccggctccggctgggacaggcctctatgacagcgtccccccctgggtccctgcgagcctctgattgggtaatactcaactgctcattttctcggccagatcgccccgctagtgttcattggttccgaaatcgcggccaaggtcgcgtgcctgttcgagaatctccacaccaccatttggcggagtcttttctttttctgcctcaggtctcccctatggactctggaccgtggggctgtattttgacatatcgggatgggtttaacgtgagtataatgtataatctcactgtcttgggtcttgagccacctacgccgctgacggtgtacgcgggagccggcagccgggttggtctgccctgcaggctgcctgcaggagtcgggacaaggtcattccttacagcaaagtggaccccgccaggtggggggcccgacctccttgtaacgggagataatggagatttcactctgagacttgaggatgtctctcaagctcaggctgggacttatacatgtcacattcacttgcaagaacagcagttgaatgcgacggttaccctggctatcataacagtaacacctaaatctttcggtagtccgggtagcctgggcaaactgttgtgtgaggtaacccccgtgtcaggtcaagagcggttcgtctggagctcattggacactccctcacagcgatcctttagcggaccctggctcgaagcccaagaagcccagctgctttcccaaccatggcagtgtcaactctatcagggtgagcgccttctcggtgcggctgtctacttcaccgaattgtcctctccgggagcgcaaagaagttgtcccagccctctgtttcccggccctagcaagcctttctgggtgctggtggtggtcggaggcgtgctggcctgctacagcctgctggtcaccgtggccttcatcatcttttgggtccgcagcaagcggagcagaggcggccacagcgactacatgaacatgacccctagacggcctggccccaccagaaagcactaccagccctacgcccctccccgggactttgccgcctacagaagc

SEQ ID NO: 160 - protein, 518 aa, Artificial Sequence
  huLag3-12aas-CD28Cys
MWEAQFLGLLFLQPLWVAPVKPLQPGAEVPVVWAQEGAPAQLPCSPTIPLQDLSLLRRAGVTWQHQPDSGPPAAAPGHPLAPGPHPAAPSSWGPRPRRYTVLSVGPGGLRSGRLPLQPRVQLDERGRQRGDFSLWLRPARRADAGEYRAAVHLRDRALSCRLRLRLGQASMTASPPGSLRASDWVILNCSFSRPDRPASVHWFRNRGQGRVPVRESPHHHLAESFLFLPQVSPMDSGPWGCILTYRDGFNVSIMYNLTVLGLEPPTPLTVYAGAGSRVGLPCRLPAGVGTRSFLTAKWTPPGGGPDLLVTGDNGDFTLRLEDVSQAQAGTYTCHIHLQEQQLNATVTLAIITVTPKSFGSPGSLGKLLCEVTPVSGQERFVWSSLDTPSQRSFSGPWLEAQEAQLLSQPWQCQLYQGERLLGAAVYFTELSSPGAQRSCPSPLFPGPSKPFWVLVVVGGVLACYSLLVTVAFIIFWVRSKRSRGGHSDYMNMTPRRPGPTRKHYQPYAPPRDFAAYRS

SEQ ID NO: 161 - DNA, 1314 bp, Artificial Sequence
  huLag3-12aas
atgtgggaagcgcagtttcttggacttctttttctccagccgctgtgggttgcgccagtaaagccgctccaacccggtgcagaggttccggtagtgtgggcgcaagagggtgcaccagcgcagctcccctgcagtccgacgattccgctgcaagatttgtcactgcttagaagggcgggcgtaacgtggcagcaccaaccggatagtggccctccggctgcagcaccagggcacccactcgcccccggccctcatcccgcagcaccgagcagctggggtcctagaccacgcagatatacagtactctcagtaggtcccggcggcctgcggtccggtcgcttgccccttcaacctagagtacagctggatgaaagaggtcgacaacggggtgatttctccctctggttgaggcctgcacgacgagcagatgctggggagtatagggctgccgtacacctgcgagaccgcgcacttagttgtagactccggctccggctgggacaggcctctatgacagcgtccccccctgggtccctgcgagcctctgattgggtaatactcaactgctcattttctcggccagatcgccccgctagtgttcattggttccgaaatcgcggccaaggtcgcgtgcctgttcgagaatctccacaccaccatttggcggagtcttttctttttctgcctcaggtctcccctatggactctggaccgtggggctgtattttgacatatcgggatgggtttaacgtgagtataatgtataatctcactgtcttgggtcttgagccacctacgccgctgacggtgtacgcgggagccggcagccgggttggtctgccctgcaggctgcctgcaggagtcgggacaaggtcattccttacagcaaagtggaccccgccaggtggggggcccgacctccttgtaacgggagataatggagatttcactctgagacttgaggatgtctctcaagctcaggctgggacttatacatgtcacattcacttgcaagaacagcagttgaatgcgacggttaccctggctatcataacagtaacacctaaatctttcggtagtccgggtagcctgggcaaactgttgtgtgaggtaacccccgtgtcaggtcaagagcggttcgtctggagctcattggacactccctcacagcgatcctttagcggaccctggctcgaagcccaagaagcccagctgctttcccaaccatggcagtgtcaactctatcagggtgagcgccttctcggtgcggctgtctacttcaccgaattgtcctctccgggagcgcaaagaagt

SEQ ID NO: 162 - protein, 438 aa, Artificial Sequence
  huLag3-12aas
MWEAQFLGLLFLQPLWVAPVKPLQPGAEVPVVWAQEGAPAQLPCSPTIPLQDLSLLRRAGVTWQHQPDSGPPAAAPGHPLAPGPHPAAPSSWGPRPRRYTVLSVGPGGLRSGRLPLQPRVQLDERGRQRGDFSLWLRPARRADAGEYRAAVHLRDRALSCRLRLRLGQASMTASPPGSLRASDWVILNCSFSRPDRPASVHWFRNRGQGRVPVRESPHHHLAESFLFLPQVSPMDSGPWGCILTYRDGFNVSIMYNLTVLGLEPPTPLTVYAGAGSRVGLPCRLPAGVGTRSFLTAKWTPPGGGPDLLVTGDNGDFTLRLEDVSQAQAGTYTCHIHLQEQQLNATVTLAIITVTPKSFGSPGSLGKLLCEVTPVSGQERFVWSSLDTPSQRSFSGPWLEAQEAQLLSQPWQCQLYQGERLLGAAVYFTELSSPGAQRS

SEQ ID NO: 163 - DNA, 1590 bp, Artificial Sequence
  huLag3-CD28Cys
atgtgggaagcgcagtttcttggacttctttttctccagccgctgtgggttgcgccagtaaagccgctccaacccggtgcagaggttccggtagtgtgggcgcaagagggtgcaccagcgcagctcccctgcagtccgacgattccgctgcaagatttgtcactgcttagaagggcgggcgtaacgtggcagcaccaaccggatagtggccctccggctgcagcaccagggcacccactcgcccccggccctcatcccgcagcaccgagcagctggggtcctagaccacgcagatatacagtactctcagtaggtcccggcggcctgcggtccggtcgcttgccccttcaacctagagtacagctggatgaaagaggtcgacaacggggtgatttctccctctggttgaggcctgcacgacgagcagatgctggggagtatagggctgccgtacacctgcgagaccgcgcacttagttgtagactccggctccggctgggacaggcctctatgacagcgtccccccctgggtccctgcgagcctctgattgggtaatactcaactgctcattttctcggccagatcgccccgctagtgttcattggttccgaaatcgcggccaaggtcgcgtgcctgttcgagaatctccacaccaccatttggcggagtcttttctttttctgcctcaggtctcccctatggactctggaccgtggggctgtattttgacatatcgggatgggtttaacgtgagtataatgtataatctcactgtcttgggtcttgagccacctacgccgctgacggtgtacgcgggagccggcagccgggttggtctgccctgcaggctgcctgcaggagtcgggacaaggtcattccttacagcaaagtggaccccgccaggtggggggcccgacctccttgtaacgggagataatggagatttcactctgagacttgaggatgtctctcaagctcaggctgggacttatacatgtcacattcacttgcaagaacagcagttgaatgcgacggttaccctggctatcataacagtaacacctaaatctttcggtagtccgggtagcctgggcaaactgttgtgtgaggtaacccccgtgtcaggtcaagagcggttcgtctggagctcattggacactccctcacagcgatcctttagcggaccctggctcgaagcccaagaagcccagctgctttcccaaccatggcagtgtcaactctatcagggtgagcgccttctcggtgcggctgtctacttcaccgaattgtcctctccgggagcgcaaagaagtggacgcgccccaggggccctcccggcaggacacctttgtcccagccctctgtttcccggccctagcaagcctttctgggtgctggtggtggtcggaggcgtgctggcctgctacagcctgctggtcaccgtggccttcatcatcttttgggtccgcagcaagcggagcagaggcggccacagcgactacatgaacatgacccctagacggcctggccccaccagaaagcactaccagccctacgcccctccccgggactttgccgcctacagaagc

SEQ ID NO: 164 - protein, 530 aa, Artificial Sequence
  huLag3-CD28Cys
MWEAQFLGLLFLQPLWVAPVKPLQPGAEVPVVWAQEGAPAQLPCSPTIPLQDLSLLRRAGVTWQHQPDSGPPAAAPGHPLAPGPHPAAPSSWGPRPRRYTVLSVGPGGLRSGRLPLQPRVQLDERGRQRGDFSLWLRPARRADAGEYRAAVHLRDRALSCRLRLRLGQASMTASPPGSLRASDWVILNCSFSRPDRPASVHWFRNRGQGRVPVRESPHHHLAESFLFLPQVSPMDSGPWGCILTYRDGFNVSIMYNLTVLGLEPPTPLTVYAGAGSRVGLPCRLPAGVGTRSFLTAKWTPPGGGPDLLVTGDNGDFTLRLEDVSQAQAGTYTCHIHLQEQQLNATVTLAIITVTPKSFGSPGSLGKLLCEVTPVSGQERFVWSSLDTPSQRSFSGPWLEAQEAQLLSQPWQCQLYQGERLLGAAVYFTELSSPGAQRSGRAPGALPAGHLCPSPLFPGPSKPFWVLVVVGGVLACYSLLVTVAFIIFWVRSKRSRGGHSDYMNMTPRRPGPTRKHYQPYAPPRDFAAYRS

SEQ ID NO: 165 - DNA, 792 bp, Artificial Sequence
  huTim3tm-CD28
atgttctcccatcttcccttcgactgtgtgttgctccttctcctcctgcttctcacccggtcaagcgaagtagagtaccgggcggaagtaggtcagaacgcatatctcccctgtttttacacacccgctgcgccgggaaacctggttcccgtgtgttggggaaagggggcatgccctgttttcgagtgtggcaacgtggtcctccggacggatgagcgagacgtgaattattggacgagcagatattggttgaatggcgattttagaaagggtgatgtgagcttgaccattgagaatgtaacgcttgctgatagcgggatatattgctgtagaattcaaatccctggtataatgaacgacgaaaaattcaatctgaagctggtaattaagccggccaaggtgacacccgccccgacacgacagcgcgacttcacggctgcctttccacgcatgttgaccacaaggggacatggtccagcggagacccagacacttggtagcctcccggacataaacctcacacaaatatccacgttggcgaacgagctccgagattccaggcttgcgaatgacctgagggattctggagctaccatcagaatcggtatctacataggtgccgggatatgcgccggtctcgcacttgccttgattttcggggcactgattcgcagcaagcggagcagaggcggccacagcgactacatgaacatgacccctagacggcctggccccaccagaaagcactaccagccctacgcccctccccgggactttgccgcctacagaagc

SEQ ID NO: 166 - protein, 264 aa, Artificial Sequence
  huTim3tm-CD28
MFSHLPFDCVLLLLLLLLTRSSEVEYRAEVGQNAYLPCFYTPAAPGNLVPVCWGKGACPVFECGNVVLRTDERDVNYWTSRYWLNGDFRKGDVSLTIENVTLADSGIYCCRIQIPGIMNDEKFNLKLVIKPAKVTPAPTRQRDFTAAFPRMLTTRGHGPAETQTLGSLPDINLTQISTLANELRDSRLANDLRDSGATIRIGIYIGAGICAGLALALIFGALIRSKRSRGGHSDYMNMTPRRPGPTRKHYQPYAPPRDFAAYRS

SEQ ID NO: 167 - DNA, 606 bp, Artificial Sequence
  huTim3 ectodomain
atgttctcccatcttcccttcgactgtgtgttgctccttctcctcctgcttctcacccggtcaagcgaagtagagtaccgggcggaagtaggtcagaacgcatatctcccctgtttttacacacccgctgcgccgggaaacctggttcccgtgtgttggggaaagggggcatgccctgttttcgagtgtggcaacgtggtcctccggacggatgagcgagacgtgaattattggacgagcagatattggttgaatggcgattttagaaagggtgatgtgagcttgaccattgagaatgtaacgcttgctgatagcgggatatattgctgtagaattcaaatccctggtataatgaacgacgaaaaattcaatctgaagctggtaattaagccggccaaggtgacacccgccccgacacgacagcgcgacttcacggctgcctttccacgcatgttgaccacaaggggacatggtccagcggagacccagacacttggtagcctcccggacataaacctcacacaaatatccacgttggcgaacgagctccgagattccaggcttgcgaatgacctgagggattctggagctaccatcagaatcggt

SEQ ID NO: 168 - protein, 202 aa, Artificial Sequence
  huTim3 ectodomain
MFSHLPFDCVLLLLLLLLTRSSEVEYRAEVGQNAYLPCFYTPAAPGNLVPVCWGKGACPVFECGNVVLRTDERDVNYWTSRYWLNGDFRKGDVSLTIENVTLADSGIYCCRIQIPGIMNDEKFNLKLVIKPAKVTPAPTRQRDFTAAFPRMLTTRGHGPAETQTLGSLPDINLTQISTLANELRDSRLANDLRDSGATIRIG

SEQ ID NO: 169 - DNA, 63 bp, Artificial Sequence
  huTim3 transmembrane
atctacataggtgccgggatatgcgccggtctcgcacttgccttgattttcggggcactgatt

SEQ ID NO: 170 - protein, 21 aa, Artificial Sequence
  huTim3 transmembrane
IYIGAGICAGLALALIFGALI

SEQ ID NO: 171 - DNA, 810 bp, Artificial Sequence
  huTim3-CD28tm
atgttctcccatcttcccttcgactgtgtgttgctccttctcctcctgcttctcacccggtcaagcgaagtagagtaccgggcggaagtaggtcagaacgcatatctcccctgtttttacacacccgctgcgccgggaaacctggttcccgtgtgttggggaaagggggcatgccctgttttcgagtgtggcaacgtggtcctccggacggatgagcgagacgtgaattattggacgagcagatattggttgaatggcgattttagaaagggtgatgtgagcttgaccattgagaatgtaacgcttgctgatagcgggatatattgctgtagaattcaaatccctggtataatgaacgacgaaaaattcaatctgaagctggtaattaagccggccaaggtgacacccgccccgacacgacagcgcgacttcacggctgcctttccacgcatgttgaccacaaggggacatggtccagcggagacccagacacttggtagcctcccggacataaacctcacacaaatatccacgttggcgaacgagctccgagattccaggcttgcgaatgacctgagggattctggagctaccatcagaatcggtttctgggtgctggtggtggtcggaggcgtgctggcctgctacagcctgctggtcaccgtggccttcatcatcttttgggtccgcagcaagcggagcagaggcggccacagcgactacatgaacatgacccctagacggcctggccccaccagaaagcactaccagccctacgcccctccccgggactttgccgcctacagaagc

SEQ ID NO: 172 - protein, 270 aa, Artificial Sequence
  huTim3-CD28tm
MFSHLPFDCVLLLLLLLLTRSSEVEYRAEVGQNAYLPCFYTPAAPGNLVPVCWGKGACPVFECGNVVLRTDERDVNYWTSRYWLNGDFRKGDVSLTIENVTLADSGIYCCRIQIPGIMNDEKFNLKLVIKPAKVTPAPTRQRDFTAAFPRMLTTRGHGPAETQTLGSLPDINLTQISTLANELRDSRLANDLRDSGATIRIGFWVLVVVGGVLACYSLLVTVAFIIFWVRSKRSRGGHSDYMNMTPRRPGPTRKHYQPYAPPRDFAAYRS

SEQ ID NO: 173 - DNA, 846 bp, Artificial Sequence
  huTim3-CD28Cys
atgttctcccatcttcccttcgactgtgtgttgctccttctcctcctgcttctcacccggtcaagcgaagtagagtaccgggcggaagtaggtcagaacgcatatctcccctgtttttacacacccgctgcgccgggaaacctggttcccgtgtgttggggaaagggggcatgccctgttttcgagtgtggcaacgtggtcctccggacggatgagcgagacgtgaattattggacgagcagatattggttgaatggcgattttagaaagggtgatgtgagcttgaccattgagaatgtaacgcttgctgatagcgggatatattgctgtagaattcaaatccctggtataatgaacgacgaaaaattcaatctgaagctggtaattaagccggccaaggtgacacccgccccgacacgacagcgcgacttcacggctgcctttccacgcatgttgaccacaaggggacatggtccagcggagacccagacacttggtagcctcccggacataaacctcacacaaatatccacgttggcgaacgagctccgagattccaggcttgcgaatgacctgagggattctggagctaccatcagaatcggttgtcccagccctctgtttcccggccctagcaagcctttctgggtgctggtggtggtcggaggcgtgctggcctgctacagcctgctggtcaccgtggccttcatcatcttttgggtccgcagcaagcggagcagaggcggccacagcgactacatgaacatgacccctagacggcctggccccaccagaaagcactaccagccctacgcccctccccgggactttgccgcctacagaagc

SEQ ID NO: 174 - protein, 282 aa, Artificial Sequence
  huTim3-CD28Cys
MFSHLPFDCVLLLLLLLLTRSSEVEYRAEVGQNAYLPCFYTPAAPGNLVPVCWGKGACPVFECGNVVLRTDERDVNYWTSRYWLNGDFRKGDVSLTIENVTLADSGIYCCRIQIPGIMNDEKFNLKLVIKPAKVTPAPTRQRDFTAAFPRMLTTRGHGPAETQTLGSLPDINLTQISTLANELRDSRLANDLRDSGATIRIGCPSPLFPGPSKPFWVLVVVGGVLACYSLLVTVAFIIFWVRSKRSRGGHSDYMNMTPRRPGPTRKHYQPYAPPRDFAAYRS

SEQ ID NO: 175 - DNA, 810 bp, Artificial Sequence
  huTim3-12aas-CD28Cys
atgttctcccatcttcccttcgactgtgtgttgctccttctcctcctgcttctcacccggtcaagcgaagtagagtaccgggcggaagtaggtcagaacgcatatctcccctgtttttacacacccgctgcgccgggaaacctggttcccgtgtgttggggaaagggggcatgccctgttttcgagtgtggcaacgtggtcctccggacggatgagcgagacgtgaattattggacgagcagatattggttgaatggcgattttagaaagggtgatgtgagcttgaccattgagaatgtaacgcttgctgatagcgggatatattgctgtagaattcaaatccctggtataatgaacgacgaaaaattcaatctgaagctggtaattaagccggccaaggtgacacccgccccgacacgacagcgcgacttcacggctgcctttccacgcatgttgaccacaaggggacatggtccagcggagacccagacacttggtagcctcccggacataaacctcacacaaatatccacgttggcgaacgagctccgagattccaggcttgcgaattgtcccagccctctgtttcccggccctagcaagcctttctgggtgctggtggtggtcggaggcgtgctggcctgctacagcctgctggtcaccgtggccttcatcatcttttgggtccgcagcaagcggagcagaggcggccacagcgactacatgaacatgacccctagacggcctggccccaccagaaagcactaccagccctacgcccctccccgggactttgccgcctacagaagc

SEQ ID NO: 176 - protein, 270 aa, Artificial Sequence
  huTim3-12aas-CD28Cys
MFSHLPFDCVLLLLLLLLTRSSEVEYRAEVGQNAYLPCFYTPAAPGNLVPVCWGKGACPVFECGNVVLRTDERDVNYWTSRYWLNGDFRKGDVSLTIENVTLADSGIYCCRIQIPGIMNDEKFNLKLVIKPAKVTPAPTRQRDFTAAFPRMLTTRGHGPAETQTLGSLPDINLTQISTLANELRDSRLANCPSPLFPGPSKPFWVLVVVGGVLACYSLLVTVAFIIFWVRSKRSRGGHSDYMNMTPRRPGPTRKHYQPYAPPRDFAAYRS

SEQ ID NO: 177 - DNA, 570 bp, Artificial Sequence
  huTim3-12aas
atgttctcccatcttcccttcgactgtgtgttgctccttctcctcctgcttctcacccggtcaagcgaagtagagtaccgggcggaagtaggtcagaacgcatatctcccctgtttttacacacccgctgcgccgggaaacctggttcccgtgtgttggggaaagggggcatgccctgttttcgagtgtggcaacgtggtcctccggacggatgagcgagacgtgaattattggacgagcagatattggttgaatggcgattttagaaagggtgatgtgagcttgaccattgagaatgtaacgcttgctgatagcgggatatattgctgtagaattcaaatccctggtataatgaacgacgaaaaattcaatctgaagctggtaattaagccggccaaggtgacacccgccccgacacgacagcgcgacttcacggctgcctttccacgcatgttgaccacaaggggacatggtccagcggagacccagacacttggtagcctcccggacataaacctcacacaaatatccacgttggcgaacgagctccgagattccaggcttgcgaat

SEQ ID NO: 178 - protein, 190 aa, Artificial Sequence
  huTim3-12aas
MFSHLPFDCVLLLLLLLLTRSSEVEYRAEVGQNAYLPCFYTPAAPGNLVPVCWGKGACPVFECGNVVLRTDERDVNYWTSRYWLNGDFRKGDVSLTIENVTLADSGIYCCRIQIPGIMNDEKFNLKLVIKPAKVTPAPTRQRDFTAAFPRMLTTRGHGPAETQTLGSLPDINLTQISTLANELRDSRLAN